European Patent Application EP 4 768 585 A1, published July 1, 2026. Title: 用于同时抑制两个靶基因表达的siRNA、药物及其应用. Applicant: 广州必贝特医药股份有限公司. Application CN. The sequence listing filed with the application follows.

SEQUENCE LISTING (713 sequences)

SEQ ID NO: 1 - RNA, 21 nt, synthetic construct
  source 1..21: mol_type = other RNA
cgagctgaacctgcaaaaatt

SEQ ID NO: 2 - RNA, 23 nt, synthetic construct
  source 1..23: mol_type = other RNA
aatttttgcaggttcagctcggt

SEQ ID NO: 3 - RNA, 21 nt, synthetic construct
  source 1..21: mol_type = other RNA
ctggagtgacatccaggacaa

SEQ ID NO: 4 - RNA, 23 nt, synthetic construct
  source 1..23: mol_type = other RNA
ttgtcctggatgtcactccagtg

SEQ ID NO: 5 - RNA, 19 nt, synthetic construct
  source 1..19: mol_type = other RNA
tgctgtgtatgatcaaaga

SEQ ID NO: 6 - RNA, 21 nt, synthetic construct
  source 1..21: mol_type = other RNA
tctttgatcatacacagcaaa

SEQ ID NO: 7 - RNA, 19 nt, synthetic construct
  source 1..19: mol_type = other RNA
cgctgtgtatgatcaaaga

SEQ ID NO: 8 - RNA, 21 nt, synthetic construct
  source 1..21: mol_type = other RNA
tctttgatcatacacagcgaa

SEQ ID NO: 9 - RNA, 21 nt, synthetic construct
  source 1..21: mol_type = other RNA
cttgctgtgtatgatcaaaga

SEQ ID NO: 10 - RNA, 21 nt, synthetic construct
  source 1..21: mol_type = other RNA
tctttgatcatacacagcaag

SEQ ID NO: 11 - RNA, 19 nt, synthetic construct
  source 1..19: mol_type = other RNA
ccattcctgtttgctgtga

SEQ ID NO: 12 - RNA, 21 nt, synthetic construct
  source 1..21: mol_type = other RNA
tcacagcaaacaggaatgggc

SEQ ID NO: 13 - RNA, 19 nt, synthetic construct
  source 1..19: mol_type = other RNA
aaaactccctcaactggaa

SEQ ID NO: 14 - RNA, 21 nt, synthetic construct
  source 1..21: mol_type = other RNA
ttccagttgagggagttttgc

SEQ ID NO: 15 - RNA, 19 nt, synthetic construct
  source 1..19: mol_type = other RNA
gaaactccctcaactggaa

SEQ ID NO: 16 - RNA, 21 nt, synthetic construct
  source 1..21: mol_type = other RNA
ttccagttgagggagtttcgc

SEQ ID NO: 17 - RNA, 22 nt, synthetic construct
  source 1..22: mol_type = other RNA
gcgaaactccctcaactggaas

SEQ ID NO: 18 - RNA, 21 nt, synthetic construct
  source 1..21: mol_type = other RNA
ttccagttgagggagtttcgc

SEQ ID NO: 19 - RNA, 21 nt, synthetic construct
  source 1..21: mol_type = other RNA
gcaaaactccctcaactggaa

SEQ ID NO: 20 - RNA, 21 nt, synthetic construct
  source 1..21: mol_type = other RNA
ttccagttgagggagttttgc

SEQ ID NO: 21 - RNA, 19 nt, synthetic construct
  source 1..19: mol_type = other RNA
gaaactccctcaactggaa

SEQ ID NO: 22 - RNA, 21 nt, synthetic construct
  source 1..21: mol_type = other RNA
ttccagttgagggagttttgg

SEQ ID NO: 23 - RNA, 21 nt, synthetic construct
  source 1..21: mol_type = other RNA
gtaaaactccctcaactggaa

SEQ ID NO: 24 - RNA, 21 nt, synthetic construct
  source 1..21: mol_type = other RNA
ttccagttgagggagttttgt

SEQ ID NO: 25 - RNA, 21 nt, synthetic construct
  source 1..21: mol_type = other RNA
ccaaaactccctcaactggaa

SEQ ID NO: 26 - RNA, 21 nt, synthetic construct
  source 1..21: mol_type = other RNA
ttccagttgagggagttttgg

SEQ ID NO: 27 - RNA, 19 nt, synthetic construct
  source 1..19: mol_type = other RNA
tccctcaactggatgaaga

SEQ ID NO: 28 - RNA, 21 nt, synthetic construct
  source 1..21: mol_type = other RNA
tcttcatccagttgagggagt

SEQ ID NO: 29 - RNA, 19 nt, synthetic construct
  source 1..19: mol_type = other RNA
catgcacagtgagctatga

SEQ ID NO: 30 - RNA, 21 nt, synthetic construct
  source 1..21: mol_type = other RNA
tcatagctcactgtgcatgtt

SEQ ID NO: 31 - RNA, 19 nt, synthetic construct
  source 1..19: mol_type = other RNA
tatatggcatgcacagtga

SEQ ID NO: 32 - RNA, 21 nt, synthetic construct
  source 1..21: mol_type = other RNA
tcactgtgcatgccatatata

SEQ ID NO: 33 - RNA, 19 nt, synthetic construct
  source 1..19: mol_type = other RNA
aagaaccagtgtttagcga

SEQ ID NO: 34 - RNA, 21 nt, synthetic construct
  source 1..21: mol_type = other RNA
tcgctaaacactggttcttgc

SEQ ID NO: 35 - RNA, 19 nt, synthetic construct
  source 1..19: mol_type = other RNA
gagaaccagtgtttagcga

SEQ ID NO: 36 - RNA, 21 nt, synthetic construct
  source 1..21: mol_type = other RNA
tcgctaaacactggttctcgc

SEQ ID NO: 37 - RNA, 21 nt, synthetic construct
  source 1..21: mol_type = other RNA
gcgagaaccagtgtttagcga

SEQ ID NO: 38 - RNA, 21 nt, synthetic construct
  source 1..21: mol_type = other RNA
tcgctaaacactggttctcgc

SEQ ID NO: 39 - RNA, 19 nt, synthetic construct
  source 1..19: mol_type = other RNA
gagaaccagtgtttagcga

SEQ ID NO: 40 - RNA, 21 nt, synthetic construct
  source 1..21: mol_type = other RNA
tcgctaaacactggttcttgg

SEQ ID NO: 41 - RNA, 21 nt, synthetic construct
  source 1..21: mol_type = other RNA
gcaagaaccagtgtttagcga

SEQ ID NO: 42 - RNA, 21 nt, synthetic construct
  source 1..21: mol_type = other RNA
tcgctaaacactggttcttgc

SEQ ID NO: 43 - RNA, 21 nt, synthetic construct
  source 1..21: mol_type = other RNA
ccaagaaccagtgtttagcga

SEQ ID NO: 44 - RNA, 21 nt, synthetic construct
  source 1..21: mol_type = other RNA
tcgctaaacactggttcttgg

SEQ ID NO: 45 - RNA, 21 nt, synthetic construct
  source 1..21: mol_type = other RNA
gtaagaaccagtgtttagcga

SEQ ID NO: 46 - RNA, 21 nt, synthetic construct
  source 1..21: mol_type = other RNA
tcgctaaacactggttcttgt

SEQ ID NO: 47 - RNA, 19 nt, synthetic construct
  source 1..19: mol_type = other RNA
gactactgttccaaaaaga

SEQ ID NO: 48 - RNA, 21 nt, synthetic construct
  source 1..21: mol_type = other RNA
tctttttggaacagtagtccc

SEQ ID NO: 49 - RNA, 19 nt, synthetic construct
  source 1..19: mol_type = other RNA
cgaccagcttgtttgtgaa

SEQ ID NO: 50 - RNA, 21 nt, synthetic construct
  source 1..21: mol_type = other RNA
ttcacaaacaagctggtcggt

SEQ ID NO: 51 - RNA, 21 nt, synthetic construct
  source 1..21: mol_type = other RNA
gccgaccagcttgtttgtgaa

SEQ ID NO: 52 - RNA, 21 nt, synthetic construct
  source 1..21: mol_type = other RNA
ttcacaaacaagctggtcggc

SEQ ID NO: 53 - RNA, 19 nt, synthetic construct
  source 1..19: mol_type = other RNA
ggaccagcttgtttgtgaa

SEQ ID NO: 54 - RNA, 21 nt, synthetic construct
  source 1..21: mol_type = other RNA
ttcacaaacaagctggtccgt

SEQ ID NO: 55 - RNA, 21 nt, synthetic construct
  source 1..21: mol_type = other RNA
gccgaccagcttgtttgtgaa

SEQ ID NO: 56 - RNA, 23 nt, synthetic construct
  source 1..23: mol_type = other RNA
ttcacaaacaagctggtcggctg

SEQ ID NO: 57 - RNA, 19 nt, synthetic construct
  source 1..19: mol_type = other RNA
ggaccagcttgtttgtgaa

SEQ ID NO: 58 - RNA, 21 nt, synthetic construct
  source 1..21: mol_type = other RNA
ttcacaaacaagctggtccgg

SEQ ID NO: 59 - RNA, 19 nt, synthetic construct
  source 1..19: mol_type = other RNA
tgaccagcttgtttgtgaa

SEQ ID NO: 60 - RNA, 21 nt, synthetic construct
  source 1..21: mol_type = other RNA
ttcacaaacaagctggtcggg

SEQ ID NO: 61 - RNA, 19 nt, synthetic construct
  source 1..19: mol_type = other RNA
tgaccagcttgtttgtgaa

SEQ ID NO: 62 - RNA, 21 nt, synthetic construct
  source 1..21: mol_type = other RNA
ttcacaaacaagctggtcgcc

SEQ ID NO: 63 - RNA, 19 nt, synthetic construct
  source 1..19: mol_type = other RNA
tgaccagcttgtttgtgaa

SEQ ID NO: 64 - RNA, 21 nt, synthetic construct
  source 1..21: mol_type = other RNA
ttcacaaacaagctggtcgtt

SEQ ID NO: 65 - RNA, 19 nt, synthetic construct
  source 1..19: mol_type = other RNA
ctgggtttattttagagaa

SEQ ID NO: 66 - RNA, 21 nt, synthetic construct
  source 1..21: mol_type = other RNA
ttctctaaaataaacccagca

SEQ ID NO: 67 - RNA, 21 nt, synthetic construct
  source 1..21: mol_type = other RNA
cgctgggtttattttagagaa

SEQ ID NO: 68 - RNA, 21 nt, synthetic construct
  source 1..21: mol_type = other RNA
ttctctaaaataaacccagcg

SEQ ID NO: 69 - RNA, 19 nt, synthetic construct
  source 1..19: mol_type = other RNA
ccgggtttattttagagaa

SEQ ID NO: 70 - RNA, 21 nt, synthetic construct
  source 1..21: mol_type = other RNA
ttctctaaaataaacccggca

SEQ ID NO: 71 - RNA, 19 nt, synthetic construct
  source 1..19: mol_type = other RNA
tcttgggcttccgtatata

SEQ ID NO: 72 - RNA, 21 nt, synthetic construct
  source 1..21: mol_type = other RNA
tatatacggaagcccaagaag

SEQ ID NO: 73 - RNA, 19 nt, synthetic construct
  source 1..19: mol_type = other RNA
cagcaaaactccctcaaca

SEQ ID NO: 74 - RNA, 21 nt, synthetic construct
  source 1..21: mol_type = other RNA
tgttgagggagttttgctgga

SEQ ID NO: 75 - RNA, 19 nt, synthetic construct
  source 1..19: mol_type = other RNA
gtctcactttccagcaaaa

SEQ ID NO: 76 - RNA, 21 nt, synthetic construct
  source 1..21: mol_type = other RNA
ttttgctggaaagtgagaccc

SEQ ID NO: 77 - RNA, 19 nt, synthetic construct
  source 1..19: mol_type = other RNA
gcctcactttccagcaaaa

SEQ ID NO: 78 - RNA, 21 nt, synthetic construct
  source 1..21: mol_type = other RNA
ttttgctggaaagtgaggccc

SEQ ID NO: 79 - RNA, 21 nt, synthetic construct
  source 1..21: mol_type = other RNA
cggtctcactttccagcaaaa

SEQ ID NO: 80 - RNA, 21 nt, synthetic construct
  source 1..21: mol_type = other RNA
ttttgctggaaagtgagaccg

SEQ ID NO: 81 - RNA, 19 nt, synthetic construct
  source 1..19: mol_type = other RNA
attcctgtttgctgtgtaa

SEQ ID NO: 82 - RNA, 21 nt, synthetic construct
  source 1..21: mol_type = other RNA
ttacacagcaaacaggaatgg

SEQ ID NO: 83 - RNA, 19 nt, synthetic construct
  source 1..19: mol_type = other RNA
gttcctgtttgctgtgtaa

SEQ ID NO: 84 - RNA, 21 nt, synthetic construct
  source 1..21: mol_type = other RNA
ttacacagcaaacaggaacgg

SEQ ID NO: 85 - RNA, 21 nt, synthetic construct
  source 1..21: mol_type = other RNA
ccactcctgtttgctgtgtaa

SEQ ID NO: 86 - RNA, 21 nt, synthetic construct
  source 1..21: mol_type = other RNA
ttacacagcaaacaggagtgg

SEQ ID NO: 87 - RNA, 21 nt, synthetic construct
  source 1..21: mol_type = other RNA
ccgttcctgtttgctgtgtaa

SEQ ID NO: 88 - RNA, 21 nt, synthetic construct
  source 1..21: mol_type = other RNA
ttacacagcaaacaggagtgg

SEQ ID NO: 89 - RNA, 21 nt, synthetic construct
  source 1..21: mol_type = other RNA
ccattcctgtttgctgtgtaa

SEQ ID NO: 90 - RNA, 21 nt, synthetic construct
  source 1..21: mol_type = other RNA
ttacacagcaaacaggaatgg

SEQ ID NO: 91 - RNA, 21 nt, synthetic construct
  source 1..21: mol_type = other RNA
ccgttcctgtttgctgtgtaa

SEQ ID NO: 92 - RNA, 21 nt, synthetic construct
  source 1..21: mol_type = other RNA
ttacacagcaaacaggaacgg

SEQ ID NO: 93 - RNA, 19 nt, synthetic construct
  source 1..19: mol_type = other RNA
actcctgtttgctgtgtaa

SEQ ID NO: 94 - RNA, 21 nt, synthetic construct
  source 1..21: mol_type = other RNA
ttacacagcaaacaggagtgg

SEQ ID NO: 95 - RNA, 21 nt, synthetic construct
  source 1..21: mol_type = other RNA
ccgttcctgtttgctgtgtaa

SEQ ID NO: 96 - RNA, 23 nt, synthetic construct
  source 1..23: mol_type = other RNA
ttacacagcaaacaggaacgggc

SEQ ID NO: 97 - RNA, 18 nt, synthetic construct
  source 1..18: mol_type = other RNA
gttcctgttgctgtgtaa

SEQ ID NO: 98 - RNA, 21 nt, synthetic construct
  source 1..21: mol_type = other RNA
ttacacagcaaacaggaacgg

SEQ ID NO: 99 - RNA, 19 nt, synthetic construct
  source 1..19: mol_type = other RNA
cttttcaagttgagaacaa

SEQ ID NO: 100 - RNA, 21 nt, synthetic construct
  source 1..21: mol_type = other RNA
ttgttctcaacttgaaaaggg

SEQ ID NO: 101 - RNA, 19 nt, synthetic construct
  source 1..19: mol_type = other RNA
gggtctcactttccagcaa

SEQ ID NO: 102 - RNA, 21 nt, synthetic construct
  source 1..21: mol_type = other RNA
ttgctggaaagtgagaccctc

SEQ ID NO: 103 - RNA, 19 nt, synthetic construct
  source 1..19: mol_type = other RNA
ggtctcactttccagcaaa

SEQ ID NO: 104 - RNA, 21 nt, synthetic construct
  source 1..21: mol_type = other RNA
tttgctggaaagtgagaccct

SEQ ID NO: 105 - RNA, 19 nt, synthetic construct
  source 1..19: mol_type = other RNA
ggtggagggtctcacttta

SEQ ID NO: 106 - RNA, 21 nt, synthetic construct
  source 1..21: mol_type = other RNA
taaagtgagaccctccacctt

SEQ ID NO: 107 - RNA, 19 nt, synthetic construct
  source 1..19: mol_type = other RNA
cgtggagggtctcacttta

SEQ ID NO: 108 - RNA, 21 nt, synthetic construct
  source 1..21: mol_type = other RNA
taaagtgagaccctccacgtt

SEQ ID NO: 109 - RNA, 21 nt, synthetic construct
  source 1..21: mol_type = other RNA
gaggtggagggtctcacttta

SEQ ID NO: 110 - RNA, 21 nt, synthetic construct
  source 1..21: mol_type = other RNA
taaagtgagaccctccacctc

SEQ ID NO: 111 - RNA, 19 nt, synthetic construct
  source 1..19: mol_type = other RNA
cccttggtctaagtgtgca

SEQ ID NO: 112 - RNA, 21 nt, synthetic construct
  source 1..21: mol_type = other RNA
tgcacacttagaccaagggga

SEQ ID NO: 113 - RNA, 21 nt, synthetic construct
  source 1..21: mol_type = other RNA
cctccttggtctaagtgtgca

SEQ ID NO: 114 - RNA, 21 nt, synthetic construct
  source 1..21: mol_type = other RNA
tgcacacttagaccaaggagg

SEQ ID NO: 115 - RNA, 19 nt, synthetic construct
  source 1..19: mol_type = other RNA
cggtctaagtgtgctgcaa

SEQ ID NO: 116 - RNA, 21 nt, synthetic construct
  source 1..21: mol_type = other RNA
ttgcagcacacttagaccgag

SEQ ID NO: 117 - RNA, 21 nt, synthetic construct
  source 1..21: mol_type = other RNA
cctggtctaagtgtgctgcaa

SEQ ID NO: 118 - RNA, 21 nt, synthetic construct
  source 1..21: mol_type = other RNA
ttgcagcacacttagaccagg

SEQ ID NO: 119 - RNA, 19 nt, synthetic construct
  source 1..19: mol_type = other RNA
ggcagccgtttctccttga

SEQ ID NO: 120 - RNA, 21 nt, synthetic construct
  source 1..21: mol_type = other RNA
tcaaggagaaacggctgcctt

SEQ ID NO: 121 - RNA, 21 nt, synthetic construct
  source 1..21: mol_type = other RNA
gaagcagccgtttctccttga

SEQ ID NO: 122 - RNA, 21 nt, synthetic construct
  source 1..21: mol_type = other RNA
tcaaggagaaacggctgcttc

SEQ ID NO: 123 - RNA, 19 nt, synthetic construct
  source 1..19: mol_type = other RNA
cctaatgagtcgactttga

SEQ ID NO: 124 - RNA, 21 nt, synthetic construct
  source 1..21: mol_type = other RNA
tcaaagtcgactcattaggag

SEQ ID NO: 125 - RNA, 21 nt, synthetic construct
  source 1..21: mol_type = other RNA
cctctaatgagtcgactttga

SEQ ID NO: 126 - RNA, 21 nt, synthetic construct
  source 1..21: mol_type = other RNA
tcaaagtcgactcattagagg

SEQ ID NO: 127 - RNA, 19 nt, synthetic construct
  source 1..19: mol_type = other RNA
gattcctgtttgctgtgta

SEQ ID NO: 128 - RNA, 21 nt, synthetic construct
  source 1..21: mol_type = other RNA
tacacagcaaacaggaatcgg

SEQ ID NO: 129 - RNA, 21 nt, synthetic construct
  source 1..21: mol_type = other RNA
gccattcctgtttgctgtgta

SEQ ID NO: 130 - RNA, 21 nt, synthetic construct
  source 1..21: mol_type = other RNA
tacacagcaaacaggaatggc

SEQ ID NO: 131 - RNA, 19 nt, synthetic construct
  source 1..19: mol_type = other RNA
ctcttctaatgagtcgaca

SEQ ID NO: 132 - RNA, 21 nt, synthetic construct
  source 1..21: mol_type = other RNA
tgtcgactcattagaagagaa

SEQ ID NO: 133 - RNA, 21 nt, synthetic construct
  source 1..21: mol_type = other RNA
ctttcttctaatgagtcgaca

SEQ ID NO: 134 - RNA, 21 nt, synthetic construct
  source 1..21: mol_type = other RNA
tgtcgactcattagaagaaag

SEQ ID NO: 135 - RNA, 19 nt, synthetic construct
  source 1..19: mol_type = other RNA
ctcttctaatgagtcgaca

SEQ ID NO: 136 - RNA, 21 nt, synthetic construct
  source 1..21: mol_type = other RNA
tgtcgactcattagaagaggg

SEQ ID NO: 137 - RNA, 21 nt, synthetic construct
  source 1..21: mol_type = other RNA
cagcgcgggactactgttcca

SEQ ID NO: 138 - RNA, 23 nt, synthetic construct
  source 1..23: mol_type = other RNA
tggaacagtagtcccgcgctgaa

SEQ ID NO: 139 - RNA, 21 nt, synthetic construct
  source 1..21: mol_type = other RNA
cagcgcgggactactgttcca

SEQ ID NO: 140 - RNA, 21 nt, synthetic construct
  source 1..21: mol_type = other RNA
tggaacagtagtcccgcgctg

SEQ ID NO: 141 - RNA, 19 nt, synthetic construct
  source 1..19: mol_type = other RNA
cactactgttccaaaaaga

SEQ ID NO: 142 - RNA, 21 nt, synthetic construct
  source 1..21: mol_type = other RNA
tctttttggaacagtagtgcc

SEQ ID NO: 143 - RNA, 21 nt, synthetic construct
  source 1..21: mol_type = other RNA
cggactactgttccaaaaaga

SEQ ID NO: 144 - RNA, 21 nt, synthetic construct
  source 1..21: mol_type = other RNA
tctttttggaacagtagtccg

SEQ ID NO: 145 - RNA, 21 nt, synthetic construct
  source 1..21: mol_type = other RNA
gcgttcccttttcaagttgaa

SEQ ID NO: 146 - RNA, 23 nt, synthetic construct
  source 1..23: mol_type = other RNA
ttcaacttgaaaagggaacgctt

SEQ ID NO: 147 - RNA, 21 nt, synthetic construct
  source 1..21: mol_type = other RNA
gcgttcccttttcaagttgaa

SEQ ID NO: 148 - RNA, 21 nt, synthetic construct
  source 1..21: mol_type = other RNA
ttcaacttgaaaagggaacgc

SEQ ID NO: 149 - RNA, 21 nt, synthetic construct
  source 1..21: mol_type = other RNA
gagtgttcccttttcaagtta

SEQ ID NO: 150 - RNA, 23 nt, synthetic construct
  source 1..23: mol_type = other RNA
taacttgaaaagggaacactctt

SEQ ID NO: 151 - RNA, 21 nt, synthetic construct
  source 1..21: mol_type = other RNA
gagtgttcccttttcaagtta

SEQ ID NO: 152 - RNA, 21 nt, synthetic construct
  source 1..21: mol_type = other RNA
taacttgaaaagggaacactc

SEQ ID NO: 153 - RNA, 19 nt, synthetic construct
  source 1..19: mol_type = other RNA
gcgttcccttttcaagtta

SEQ ID NO: 154 - RNA, 21 nt, synthetic construct
  source 1..21: mol_type = other RNA
taacttgaaaagggaacgctt

SEQ ID NO: 155 - RNA, 19 nt, synthetic construct
  source 1..19: mol_type = other RNA
ttttgagcttgaagcggaa

SEQ ID NO: 156 - RNA, 21 nt, synthetic construct
  source 1..21: mol_type = other RNA
ttccgcttcaagctcaaaagg

SEQ ID NO: 157 - RNA, 21 nt, synthetic construct
  source 1..21: mol_type = other RNA
ctttttgagcttgaagcggaa

SEQ ID NO: 158 - RNA, 21 nt, synthetic construct
  source 1..21: mol_type = other RNA
ttccgcttcaagctcaaaaag

SEQ ID NO: 159 - RNA, 19 nt, synthetic construct
  source 1..19: mol_type = other RNA
cgcaaaaattgagcaatga

SEQ ID NO: 160 - RNA, 21 nt, synthetic construct
  source 1..21: mol_type = other RNA
tcattgctcaatttttgcggg

SEQ ID NO: 161 - RNA, 19 nt, synthetic construct
  source 1..19: mol_type = other RNA
gctttgagctggaaagcaa

SEQ ID NO: 162 - RNA, 21 nt, synthetic construct
  source 1..21: mol_type = other RNA
ttgctttccagctcaaagtgg

SEQ ID NO: 163 - RNA, 19 nt, synthetic construct
  source 1..19: mol_type = other RNA
ctttcaagttgagaacaaa

SEQ ID NO: 164 - RNA, 21 nt, synthetic construct
  source 1..21: mol_type = other RNA
tttgttctcaacttgaaaggg

SEQ ID NO: 165 - RNA, 21 nt, synthetic construct
  source 1..21: mol_type = other RNA
ccctttcaagttgagaacaaa

SEQ ID NO: 166 - RNA, 21 nt, synthetic construct
  source 1..21: mol_type = other RNA
tttgttctcaacttgaaaggg

SEQ ID NO: 167 - RNA, 19 nt, synthetic construct
  source 1..19: mol_type = other RNA
ccttcaagttgagaacaaa

SEQ ID NO: 168 - RNA, 19 nt, synthetic construct
  source 1..19: mol_type = other RNA
tttgttctcaacttgaagg

SEQ ID NO: 169 - RNA, 19 nt, synthetic construct
  source 1..19: mol_type = other RNA
ctcggtttgtatttagtga

SEQ ID NO: 170 - RNA, 21 nt, synthetic construct
  source 1..21: mol_type = other RNA
tcactaaatacaaaccgaggg

SEQ ID NO: 171 - RNA, 19 nt, synthetic construct
  source 1..19: mol_type = other RNA
gccttcggtttgtatttaa

SEQ ID NO: 172 - RNA, 21 nt, synthetic construct
  source 1..21: mol_type = other RNA
ttaaatacaaaccgaaggcgg

SEQ ID NO: 173 - RNA, 19 nt, synthetic construct
  source 1..19: mol_type = other RNA
gcattgccttcggtttgta

SEQ ID NO: 174 - RNA, 21 nt, synthetic construct
  source 1..21: mol_type = other RNA
tacaaaccgaaggcaatgcgg

SEQ ID NO: 175 - RNA, 21 nt, synthetic construct
  source 1..21: mol_type = other RNA
ctgcattgccttcggtttgta

SEQ ID NO: 176 - RNA, 21 nt, synthetic construct
  source 1..21: mol_type = other RNA
tacaaaccgaaggcaatgcag

SEQ ID NO: 177 - RNA, 19 nt, synthetic construct
  source 1..19: mol_type = other RNA
ctgtgttagtaataaacga

SEQ ID NO: 178 - RNA, 21 nt, synthetic construct
  source 1..21: mol_type = other RNA
tcgtttattactaacacaggg

SEQ ID NO: 179 - RNA, 19 nt, synthetic construct
  source 1..19: mol_type = other RNA
gcggaaccatagctggtta

SEQ ID NO: 180 - RNA, 21 nt, synthetic construct
  source 1..21: mol_type = other RNA
taaccagctatggttccgcgg

SEQ ID NO: 181 - RNA, 19 nt, synthetic construct
  source 1..19: mol_type = other RNA
cccgtgtagtgtctgtaaa

SEQ ID NO: 182 - RNA, 21 nt, synthetic construct
  source 1..21: mol_type = other RNA
tttacagacactacacggggg

SEQ ID NO: 183 - RNA, 19 nt, synthetic construct
  source 1..19: mol_type = other RNA
gcgaccagcttgtttgtga

SEQ ID NO: 184 - RNA, 21 nt, synthetic construct
  source 1..21: mol_type = other RNA
tcacaaacaagctggtcgctt

SEQ ID NO: 185 - RNA, 19 nt, synthetic construct
  source 1..19: mol_type = other RNA
gcggacaaatcagcgatga

SEQ ID NO: 186 - RNA, 21 nt, synthetic construct
  source 1..21: mol_type = other RNA
tcatcgctgatttgtccgcgg

SEQ ID NO: 187 - RNA, 19 nt, synthetic construct
  source 1..19: mol_type = other RNA
cctaatgagtcgactttga

SEQ ID NO: 188 - RNA, 21 nt, synthetic construct
  source 1..21: mol_type = other RNA
tcaaagtcgactcattagggg

SEQ ID NO: 189 - RNA, 19 nt, synthetic construct
  source 1..19: mol_type = other RNA
cgctgtgtatgatcaaaga

SEQ ID NO: 190 - RNA, 21 nt, synthetic construct
  source 1..21: mol_type = other RNA
tctttgatcatacacagcggg

SEQ ID NO: 191 - RNA, 19 nt, synthetic construct
  source 1..19: mol_type = other RNA
cttttgagcttgaagcgga

SEQ ID NO: 192 - RNA, 21 nt, synthetic construct
  source 1..21: mol_type = other RNA
tccgcttcaagctcaaaaggg

SEQ ID NO: 193 - RNA, 19 nt, synthetic construct
  source 1..19: mol_type = other RNA
gcgaggatcttatgaccta

SEQ ID NO: 194 - RNA, 21 nt, synthetic construct
  source 1..21: mol_type = other RNA
taggtcataagatccttgcgg

SEQ ID NO: 195 - RNA, 19 nt, synthetic construct
  source 1..19: mol_type = other RNA
aactggtgctgcaaggata

SEQ ID NO: 196 - RNA, 21 nt, synthetic construct
  source 1..21: mol_type = other RNA
tatccttgcagcaccagttgg

SEQ ID NO: 197 - RNA, 19 nt, synthetic construct
  source 1..19: mol_type = other RNA
cgctgggtttattttagaa

SEQ ID NO: 198 - RNA, 21 nt, synthetic construct
  source 1..21: mol_type = other RNA
ttctaaaataaacccagcggg

SEQ ID NO: 199 - RNA, 19 nt, synthetic construct
  source 1..19: mol_type = other RNA
gcccattcctgtttgctga

SEQ ID NO: 200 - RNA, 21 nt, synthetic construct
  source 1..21: mol_type = other RNA
tcagcaaacaggaatgggcgg

SEQ ID NO: 201 - RNA, 19 nt, synthetic construct
  source 1..19: mol_type = other RNA
gaccgcccattcctgttta

SEQ ID NO: 202 - RNA, 21 nt, synthetic construct
  source 1..21: mol_type = other RNA
taaacaggaatgggcggttgg

SEQ ID NO: 203 - RNA, 19 nt, synthetic construct
  source 1..19: mol_type = other RNA
gagtgcccttcactgagaa

SEQ ID NO: 204 - RNA, 21 nt, synthetic construct
  source 1..21: mol_type = other RNA
ttctcagtgaagggcacttgg

SEQ ID NO: 205 - RNA, 19 nt, synthetic construct
  source 1..19: mol_type = other RNA
gcttctcggtgactcaaga

SEQ ID NO: 206 - RNA, 21 nt, synthetic construct
  source 1..21: mol_type = other RNA
tcttgagtcaccgagaagtgg

SEQ ID NO: 207 - RNA, 19 nt, synthetic construct
  source 1..19: mol_type = other RNA
gtggcaggatggaagacta

SEQ ID NO: 208 - RNA, 21 nt, synthetic construct
  source 1..21: mol_type = other RNA
tagtcttccatcctgtcacgg

SEQ ID NO: 209 - RNA, 19 nt, synthetic construct
  source 1..19: mol_type = other RNA
accccgtcatccacaatga

SEQ ID NO: 210 - RNA, 21 nt, synthetic construct
  source 1..21: mol_type = other RNA
tcattgtggatgacggggtgg

SEQ ID NO: 211 - RNA, 19 nt, synthetic construct
  source 1..19: mol_type = other RNA
gaccccaccttcataccta

SEQ ID NO: 212 - RNA, 21 nt, synthetic construct
  source 1..21: mol_type = other RNA
taggtatgaaggtggggtctt

SEQ ID NO: 213 - RNA, 19 nt, synthetic construct
  source 1..19: mol_type = other RNA
gtctggacttcacagaaca

SEQ ID NO: 214 - RNA, 21 nt, synthetic construct
  source 1..21: mol_type = other RNA
tgttctgtgaagtccagacgg

SEQ ID NO: 215 - RNA, 19 nt, synthetic construct
  source 1..19: mol_type = other RNA
ccgcaaaaattgagcaata

SEQ ID NO: 216 - RNA, 21 nt, synthetic construct
  source 1..21: mol_type = other RNA
tattgctcaatttttgcgggt

SEQ ID NO: 217 - RNA, 19 nt, synthetic construct
  source 1..19: mol_type = other RNA
cgaagcggatgagagagaa

SEQ ID NO: 218 - RNA, 21 nt, synthetic construct
  source 1..21: mol_type = other RNA
ttctctctcatccgcttcggg

SEQ ID NO: 219 - RNA, 19 nt, synthetic construct
  source 1..19: mol_type = other RNA
cgagtcgactttgagctga

SEQ ID NO: 220 - RNA, 21 nt, synthetic construct
  source 1..21: mol_type = other RNA
tcagctcaaagtcgactcgtt

SEQ ID NO: 221 - RNA, 19 nt, synthetic construct
  source 1..19: mol_type = other RNA
cggtctaagtgtgctgcaa

SEQ ID NO: 222 - RNA, 21 nt, synthetic construct
  source 1..21: mol_type = other RNA
ttgcagcacacttagaccggg

SEQ ID NO: 223 - RNA, 19 nt, synthetic construct
  source 1..19: mol_type = other RNA
gctcccttttcaagttgaa

SEQ ID NO: 224 - RNA, 21 nt, synthetic construct
  source 1..21: mol_type = other RNA
ttcaacttgaaaagggagcgg

SEQ ID NO: 225 - RNA, 19 nt, synthetic construct
  source 1..19: mol_type = other RNA
ctccacagatgcttgtgaa

SEQ ID NO: 226 - RNA, 21 nt, synthetic construct
  source 1..21: mol_type = other RNA
ttcacaagcatctgtggaggg

SEQ ID NO: 227 - RNA, 19 nt, synthetic construct
  source 1..19: mol_type = other RNA
cgtgatttttgaacaataa

SEQ ID NO: 228 - RNA, 21 nt, synthetic construct
  source 1..21: mol_type = other RNA
ttattgttcaaaaatcacggg

SEQ ID NO: 229 - RNA, 19 nt, synthetic construct
  source 1..19: mol_type = other RNA
ggatttctgtttgaatgca

SEQ ID NO: 230 - RNA, 21 nt, synthetic construct
  source 1..21: mol_type = other RNA
tgcattcaaacagaaattcgg

SEQ ID NO: 231 - RNA, 19 nt, synthetic construct
  source 1..19: mol_type = other RNA
gaccagcttgtttgtgaaa

SEQ ID NO: 232 - RNA, 21 nt, synthetic construct
  source 1..21: mol_type = other RNA
tttcacaaacaagctggtcgg

SEQ ID NO: 233 - RNA, 19 nt, synthetic construct
  source 1..19: mol_type = other RNA
accagcttgtttgtgaaaa

SEQ ID NO: 234 - RNA, 21 nt, synthetic construct
  source 1..21: mol_type = other RNA
ttttcacaaacaagctggtcg

SEQ ID NO: 235 - RNA, 19 nt, synthetic construct
  source 1..19: mol_type = other RNA
accgaccagcttgtttgta

SEQ ID NO: 236 - RNA, 21 nt, synthetic construct
  source 1..21: mol_type = other RNA
tacaaacaagctggtcggttg

SEQ ID NO: 237 - RNA, 21 nt, synthetic construct
  source 1..21: mol_type = other RNA
ctccgtatatatggcatgcaa

SEQ ID NO: 238 - RNA, 21 nt, synthetic construct
  source 1..21: mol_type = other RNA
ttgcatgccatatatacggag

SEQ ID NO: 239 - RNA, 19 nt, synthetic construct
  source 1..19: mol_type = other RNA
ccgtatatatggcatgcaa

SEQ ID NO: 240 - RNA, 21 nt, synthetic construct
  source 1..21: mol_type = other RNA
ttgcatgccatatatacgggg

SEQ ID NO: 241 - RNA, 19 nt, synthetic construct
  source 1..19: mol_type = other RNA
agttctgggtggacaacaa

SEQ ID NO: 242 - RNA, 21 nt, synthetic construct
  source 1..21: mol_type = other RNA
ttgttgtccacccagaacttt

SEQ ID NO: 243 - RNA, 19 nt, synthetic construct
  source 1..19: mol_type = other RNA
cgcattgccttcggtttga

SEQ ID NO: 244 - RNA, 21 nt, synthetic construct
  source 1..21: mol_type = other RNA
tcaaaccgaaggcaatgcggg

SEQ ID NO: 245 - RNA, 21 nt, synthetic construct
  source 1..21: mol_type = other RNA
cttgcattgccttcggtttga

SEQ ID NO: 246 - RNA, 21 nt, synthetic construct
  source 1..21: mol_type = other RNA
tcaaaccgaaggcaatgcaag

SEQ ID NO: 247 - RNA, 21 nt, synthetic construct
  source 1..21: mol_type = other RNA
gcgttcccttttcaagttgaa

SEQ ID NO: 248 - RNA, 21 nt, synthetic construct
  source 1..21: mol_type = other RNA
ttcaacttgaaaagggaacgc

SEQ ID NO: 249 - RNA, 21 nt, synthetic construct
  source 1..21: mol_type = other RNA
agtgttcccttttcaagttga

SEQ ID NO: 250 - RNA, 21 nt, synthetic construct
  source 1..21: mol_type = other RNA
tcaacttgaaaagggaacact

SEQ ID NO: 251 - RNA, 21 nt, synthetic construct
  source 1..21: mol_type = other RNA
ctttctagacctgttttgcta

SEQ ID NO: 252 - RNA, 21 nt, synthetic construct
  source 1..21: mol_type = other RNA
tagcaaaacaggtctagaaag

SEQ ID NO: 253 - RNA, 21 nt, synthetic construct
  source 1..21: mol_type = other RNA
ctacagccaacttttctagaa

SEQ ID NO: 254 - RNA, 21 nt, synthetic construct
  source 1..21: mol_type = other RNA
ttctagaaaagttggctgtag

SEQ ID NO: 255 - RNA, 19 nt, synthetic construct
  source 1..19: mol_type = other RNA
acagccaacttttctagaa

SEQ ID NO: 256 - RNA, 21 nt, synthetic construct
  source 1..21: mol_type = other RNA
ttctagaaaagttggctgtaa

SEQ ID NO: 257 - RNA, 19 nt, synthetic construct
  source 1..19: mol_type = other RNA
gcagccaacttttctagaa

SEQ ID NO: 258 - RNA, 21 nt, synthetic construct
  source 1..21: mol_type = other RNA
ttctagaaaagttggctgcaa

SEQ ID NO: 259 - RNA, 19 nt, synthetic construct
  source 1..19: mol_type = other RNA
gcagccaacttttctagaa

SEQ ID NO: 260 - RNA, 21 nt, synthetic construct
  source 1..21: mol_type = other RNA
ttctagaaaagttggctgtgg

SEQ ID NO: 261 - RNA, 21 nt, synthetic construct
  source 1..21: mol_type = other RNA
cctgggttttgtagcatttta

SEQ ID NO: 262 - RNA, 21 nt, synthetic construct
  source 1..21: mol_type = other RNA
taaaatgctacaaaacccagg

SEQ ID NO: 263 - RNA, 19 nt, synthetic construct
  source 1..19: mol_type = other RNA
cgggttttgtagcatttta

SEQ ID NO: 264 - RNA, 21 nt, synthetic construct
  source 1..21: mol_type = other RNA
taaaatgctacaaaacccggg

SEQ ID NO: 265 - RNA, 19 nt, synthetic construct
  source 1..19: mol_type = other RNA
ctttgtaacttgaagataa

SEQ ID NO: 266 - RNA, 21 nt, synthetic construct
  source 1..21: mol_type = other RNA
ttatcttcaagttacaaaggc

SEQ ID NO: 267 - RNA, 21 nt, synthetic construct
  source 1..21: mol_type = other RNA
gcctttgtaacttgaagataa

SEQ ID NO: 268 - RNA, 21 nt, synthetic construct
  source 1..21: mol_type = other RNA
ttatcttcaagttacaaaggc

SEQ ID NO: 269 - RNA, 21 nt, synthetic construct
  source 1..21: mol_type = other RNA
ccgttgcctttttacagccaa

SEQ ID NO: 270 - RNA, 21 nt, synthetic construct
  source 1..21: mol_type = other RNA
ttggctgtaaaaaggcaacgg

SEQ ID NO: 271 - RNA, 21 nt, synthetic construct
  source 1..21: mol_type = other RNA
cctgttgcctttttacagcca

SEQ ID NO: 272 - RNA, 21 nt, synthetic construct
  source 1..21: mol_type = other RNA
tggctgtaaaaaggcaacagg

SEQ ID NO: 273 - RNA, 19 nt, synthetic construct
  source 1..19: mol_type = other RNA
cttgtaacttgaagatata

SEQ ID NO: 274 - RNA, 21 nt, synthetic construct
  source 1..21: mol_type = other RNA
tatatcttcaagttacaagag

SEQ ID NO: 275 - RNA, 21 nt, synthetic construct
  source 1..21: mol_type = other RNA
cctttgtaacttgaagatata

SEQ ID NO: 276 - RNA, 21 nt, synthetic construct
  source 1..21: mol_type = other RNA
tatatcttcaagttacaaagg

SEQ ID NO: 277 - RNA, 21 nt, synthetic construct
  source 1..21: mol_type = other RNA
cccttgtaacttgaagatata

SEQ ID NO: 278 - RNA, 21 nt, synthetic construct
  source 1..21: mol_type = other RNA
tatatcttcaagttacaaggg

SEQ ID NO: 279 - RNA, 19 nt, synthetic construct
  source 1..19: mol_type = other RNA
cctgtaacttgaagatata

SEQ ID NO: 280 - RNA, 21 nt, synthetic construct
  source 1..21: mol_type = other RNA
tatatcttcaagttacagggg

SEQ ID NO: 281 - RNA, 19 nt, synthetic construct
  source 1..19: mol_type = other RNA
ctgaagatatttattctga

SEQ ID NO: 282 - RNA, 21 nt, synthetic construct
  source 1..21: mol_type = other RNA
tcagaataaatatcttcaggt

SEQ ID NO: 283 - RNA, 21 nt, synthetic construct
  source 1..21: mol_type = other RNA
gcttgaagatatttattctga

SEQ ID NO: 284 - RNA, 21 nt, synthetic construct
  source 1..21: mol_type = other RNA
tcagaataaatatcttcaagc

SEQ ID NO: 285 - DNA, 21 bp, synthetic construct
  source 1..21: mol_type = other DNA
gcttgaagatatttattctga

SEQ ID NO: 286 - RNA, 21 nt, synthetic construct
  source 1..21: mol_type = other RNA
tgtctagaaaagttggctgtg

SEQ ID NO: 287 - RNA, 19 nt, synthetic construct
  source 1..19: mol_type = other RNA
cctgttgcctttttacaga

SEQ ID NO: 288 - RNA, 21 nt, synthetic construct
  source 1..21: mol_type = other RNA
tctgtaaaaaggcaacaggga

SEQ ID NO: 289 - RNA, 21 nt, synthetic construct
  source 1..21: mol_type = other RNA
cctctgttgcctttttacaga

SEQ ID NO: 290 - RNA, 21 nt, synthetic construct
  source 1..21: mol_type = other RNA
tctgtaaaaaggcaacagagg

SEQ ID NO: 291 - RNA, 19 nt, synthetic construct
  source 1..19: mol_type = other RNA
cgtcctctctgttgcctta

SEQ ID NO: 292 - RNA, 21 nt, synthetic construct
  source 1..21: mol_type = other RNA
taaggcaacagagaggacgga

SEQ ID NO: 293 - RNA, 21 nt, synthetic construct
  source 1..21: mol_type = other RNA
cctgtcctctctgttgcctta

SEQ ID NO: 294 - RNA, 21 nt, synthetic construct
  source 1..21: mol_type = other RNA
taaggcaacagagaggacagg

SEQ ID NO: 295 - RNA, 19 nt, synthetic construct
  source 1..19: mol_type = other RNA
cggcggagatgcttctaaa

SEQ ID NO: 296 - RNA, 21 nt, synthetic construct
  source 1..21: mol_type = other RNA
tttagaagcatctccgccggg

SEQ ID NO: 297 - RNA, 21 nt, synthetic construct
  source 1..21: mol_type = other RNA
cccggcggagatgcttctaaa

SEQ ID NO: 298 - RNA, 21 nt, synthetic construct
  source 1..21: mol_type = other RNA
tttagaagcatctccgccggg

SEQ ID NO: 299 - RNA, 19 nt, synthetic construct
  source 1..19: mol_type = other RNA
ggcagacatttatctttta

SEQ ID NO: 300 - RNA, 21 nt, synthetic construct
  source 1..21: mol_type = other RNA
taaaagataaatgtctgcctg

SEQ ID NO: 301 - RNA, 21 nt, synthetic construct
  source 1..21: mol_type = other RNA
cgagcagacatttatctttta

SEQ ID NO: 302 - RNA, 21 nt, synthetic construct
  source 1..21: mol_type = other RNA
taaaagataaatgtctgctcg

SEQ ID NO: 303 - RNA, 21 nt, synthetic construct
  source 1..21: mol_type = other RNA
ggcatggaactttttccgtta

SEQ ID NO: 304 - RNA, 21 nt, synthetic construct
  source 1..21: mol_type = other RNA
taacggaaaaagttccatgcc

SEQ ID NO: 305 - RNA, 19 nt, synthetic construct
  source 1..19: mol_type = other RNA
ccgcaggcatggaacttta

SEQ ID NO: 306 - RNA, 21 nt, synthetic construct
  source 1..21: mol_type = other RNA
taaagttccatgcctgcgggc

SEQ ID NO: 307 - RNA, 21 nt, synthetic construct
  source 1..21: mol_type = other RNA
ccctgcaggcatggaacttta

SEQ ID NO: 308 - RNA, 21 nt, synthetic construct
  source 1..21: mol_type = other RNA
taaagttccatgcctgcaggg

SEQ ID NO: 309 - RNA, 21 nt, synthetic construct
  source 1..21: mol_type = other RNA
gccaacttttctagacctgta

SEQ ID NO: 310 - RNA, 21 nt, synthetic construct
  source 1..21: mol_type = other RNA
tacaggtctagaaaagttggc

SEQ ID NO: 311 - RNA, 21 nt, synthetic construct
  source 1..21: mol_type = other RNA
gagccaacttttctagaccta

SEQ ID NO: 312 - RNA, 21 nt, synthetic construct
  source 1..21: mol_type = other RNA
taggtctagaaaagttggctc

SEQ ID NO: 313 - RNA, 21 nt, synthetic construct
  source 1..21: mol_type = other RNA
gcagccaacttttctagacca

SEQ ID NO: 314 - RNA, 23 nt, synthetic construct
  source 1..23: mol_type = other RNA
tggtctagaaaagttggctgcgg

SEQ ID NO: 315 - RNA, 21 nt, synthetic construct
  source 1..21: mol_type = other RNA
cgttgcctttttacagccaaa

SEQ ID NO: 316 - RNA, 21 nt, synthetic construct
  source 1..21: mol_type = other RNA
tttggctgtaaaaaggcaacg

SEQ ID NO: 317 - RNA, 21 nt, synthetic construct
  source 1..21: mol_type = other RNA
ccctgttgcctttttacagca

SEQ ID NO: 318 - RNA, 21 nt, synthetic construct
  source 1..21: mol_type = other RNA
tgctgtaaaaaggcaacaggg

SEQ ID NO: 319 - RNA, 21 nt, synthetic construct
  source 1..21: mol_type = other RNA
cgtcctctctgttgcctttta

SEQ ID NO: 320 - RNA, 21 nt, synthetic construct
  source 1..21: mol_type = other RNA
taaaaggcaacagagaggacg

SEQ ID NO: 321 - RNA, 19 nt, synthetic construct
  source 1..19: mol_type = other RNA
ccctctctgttgcctttta

SEQ ID NO: 322 - RNA, 21 nt, synthetic construct
  source 1..21: mol_type = other RNA
taaaaggcaacagagagggca

SEQ ID NO: 323 - RNA, 19 nt, synthetic construct
  source 1..19: mol_type = other RNA
cgaagatatttattctgga

SEQ ID NO: 324 - RNA, 21 nt, synthetic construct
  source 1..21: mol_type = other RNA
tccagaataaatatcttcgag

SEQ ID NO: 325 - RNA, 21 nt, synthetic construct
  source 1..21: mol_type = other RNA
cctgaagatatttattctgga

SEQ ID NO: 326 - RNA, 21 nt, synthetic construct
  source 1..21: mol_type = other RNA
tccagaataaatatcttcagg

SEQ ID NO: 327 - RNA, 19 nt, synthetic construct
  source 1..19: mol_type = other RNA
cgggcagaatgacttttaa

SEQ ID NO: 328 - RNA, 21 nt, synthetic construct
  source 1..21: mol_type = other RNA
ttaaaagtcattctgcccgcg

SEQ ID NO: 329 - RNA, 21 nt, synthetic construct
  source 1..21: mol_type = other RNA
cgcgggcagaatgacttttaa

SEQ ID NO: 330 - RNA, 21 nt, synthetic construct
  source 1..21: mol_type = other RNA
ttaaaagtcattctgcccgcg

SEQ ID NO: 331 - RNA, 21 nt, synthetic construct
  source 1..21: mol_type = other RNA
cgtggggcatttcaccattca

SEQ ID NO: 332 - RNA, 21 nt, synthetic construct
  source 1..21: mol_type = other RNA
tgaatggtgaaatgccccacg

SEQ ID NO: 333 - RNA, 19 nt, synthetic construct
  source 1..19: mol_type = other RNA
ctgggtctgtcctctctga

SEQ ID NO: 334 - RNA, 21 nt, synthetic construct
  source 1..21: mol_type = other RNA
tcagagaggacagacccagaa

SEQ ID NO: 335 - RNA, 21 nt, synthetic construct
  source 1..21: mol_type = other RNA
ctttgggtctgtcctctctga

SEQ ID NO: 336 - RNA, 21 nt, synthetic construct
  source 1..21: mol_type = other RNA
tcagagaggacagacccaaag

SEQ ID NO: 337 - RNA, 19 nt, synthetic construct
  source 1..19: mol_type = other RNA
cggagtttattcggaaaaa

SEQ ID NO: 338 - RNA, 21 nt, synthetic construct
  source 1..21: mol_type = other RNA
tttttccgaataaactccggg

SEQ ID NO: 339 - RNA, 21 nt, synthetic construct
  source 1..21: mol_type = other RNA
cccggagtttattcggaaaaa

SEQ ID NO: 340 - RNA, 21 nt, synthetic construct
  source 1..21: mol_type = other RNA
tttttccgaataaactccggg

SEQ ID NO: 341 - RNA, 19 nt, synthetic construct
  source 1..19: mol_type = other RNA
gtagacatttatcttttga

SEQ ID NO: 342 - RNA, 21 nt, synthetic construct
  source 1..21: mol_type = other RNA
tcaaaagataaatgtctgttt

SEQ ID NO: 343 - RNA, 21 nt, synthetic construct
  source 1..21: mol_type = other RNA
gagcagacatttatcttttga

SEQ ID NO: 344 - RNA, 21 nt, synthetic construct
  source 1..21: mol_type = other RNA
tcaaaagataaatgtctgctc

SEQ ID NO: 345 - RNA, 21 nt, synthetic construct
  source 1..21: mol_type = other RNA
cctgccaaagatgtcatcaaa

SEQ ID NO: 346 - RNA, 23 nt, synthetic construct
  source 1..23: mol_type = other RNA
tttgatgacatctttggcaggga

SEQ ID NO: 347 - RNA, 21 nt, synthetic construct
  source 1..21: mol_type = other RNA
ctaatggaggcttagctttca

SEQ ID NO: 348 - RNA, 23 nt, synthetic construct
  source 1..23: mol_type = other RNA
tgaaagctaagcctccattagtc

SEQ ID NO: 349 - RNA, 21 nt, synthetic construct
  source 1..21: mol_type = other RNA
caatggaggcttagctttcta

SEQ ID NO: 350 - RNA, 23 nt, synthetic construct
  source 1..23: mol_type = other RNA
tagaaagctaagcctccattgat

SEQ ID NO: 351 - RNA, 21 nt, synthetic construct
  source 1..21: mol_type = other RNA
cgatccacttctctgccaaaa

SEQ ID NO: 352 - RNA, 23 nt, synthetic construct
  source 1..23: mol_type = other RNA
ttttggcagagaagtggatcggt

SEQ ID NO: 353 - RNA, 19 nt, synthetic construct
  source 1..19: mol_type = other RNA
gttgagctttaaaatggta

SEQ ID NO: 354 - RNA, 21 nt, synthetic construct
  source 1..21: mol_type = other RNA
taccattttaaagctcagctt

SEQ ID NO: 355 - RNA, 21 nt, synthetic construct
  source 1..21: mol_type = other RNA
cggctgagctttaaaatggta

SEQ ID NO: 356 - RNA, 21 nt, synthetic construct
  source 1..21: mol_type = other RNA
taccattttaaagctcagccg

SEQ ID NO: 357 - RNA, 19 nt, synthetic construct
  source 1..19: mol_type = other RNA
cggaatgacttttattgaa

SEQ ID NO: 358 - RNA, 21 nt, synthetic construct
  source 1..21: mol_type = other RNA
ttcaataaaagtcattctgtt

SEQ ID NO: 359 - RNA, 21 nt, synthetic construct
  source 1..21: mol_type = other RNA
cgcagaatgacttttattgaa

SEQ ID NO: 360 - RNA, 21 nt, synthetic construct
  source 1..21: mol_type = other RNA
ttcaataaaagtcattctgcg

SEQ ID NO: 361 - RNA, 19 nt, synthetic construct
  source 1..19: mol_type = other RNA
cgacttttattgagctcta

SEQ ID NO: 362 - RNA, 21 nt, synthetic construct
  source 1..21: mol_type = other RNA
tagagctcaataaaagtcgtt

SEQ ID NO: 363 - RNA, 21 nt, synthetic construct
  source 1..21: mol_type = other RNA
gatgacttttattgagctcta

SEQ ID NO: 364 - RNA, 21 nt, synthetic construct
  source 1..21: mol_type = other RNA
tagagctcaataaaagtcatc

SEQ ID NO: 365 - RNA, 21 nt, synthetic construct
  source 1..21: mol_type = other RNA
ctttattgagctcttgttcca

SEQ ID NO: 366 - RNA, 23 nt, synthetic construct
  source 1..23: mol_type = other RNA
tggaacaagagctcaataaaggt

SEQ ID NO: 367 - RNA, 19 nt, synthetic construct
  source 1..19: mol_type = other RNA
cgggattcttcccatggaa

SEQ ID NO: 368 - RNA, 21 nt, synthetic construct
  source 1..21: mol_type = other RNA
ttccatgggaagaatcctgtt

SEQ ID NO: 369 - RNA, 21 nt, synthetic construct
  source 1..21: mol_type = other RNA
cgcaggattcttcccatggaa

SEQ ID NO: 370 - RNA, 21 nt, synthetic construct
  source 1..21: mol_type = other RNA
ttccatgggaagaatcctgcg

SEQ ID NO: 371 - RNA, 21 nt, synthetic construct
  source 1..21: mol_type = other RNA
cgagccacctttactctgcta

SEQ ID NO: 372 - RNA, 21 nt, synthetic construct
  source 1..21: mol_type = other RNA
tagcagagtaaaggtggctcg

SEQ ID NO: 373 - RNA, 21 nt, synthetic construct
  source 1..21: mol_type = other RNA
cccctgattaatggaggctta

SEQ ID NO: 374 - RNA, 23 nt, synthetic construct
  source 1..23: mol_type = other RNA
taagcctccattaatcagggggc

SEQ ID NO: 375 - RNA, 21 nt, synthetic construct
  source 1..21: mol_type = other RNA
cttattctgggttttgtagca

SEQ ID NO: 376 - RNA, 21 nt, synthetic construct
  source 1..21: mol_type = other RNA
tgctacaaaacccagaataag

SEQ ID NO: 377 - RNA, 19 nt, synthetic construct
  source 1..19: mol_type = other RNA
cattctgggttttgtagca

SEQ ID NO: 378 - RNA, 21 nt, synthetic construct
  source 1..21: mol_type = other RNA
tgctacaaaacccagaatgaa

SEQ ID NO: 379 - RNA, 19 nt, synthetic construct
  source 1..19: mol_type = other RNA
cattctgggttttgtagca

SEQ ID NO: 380 - RNA, 21 nt, synthetic construct
  source 1..21: mol_type = other RNA
tgctacaaaacccagaatggg

SEQ ID NO: 381 - RNA, 19 nt, synthetic construct
  source 1..19: mol_type = other RNA
tattctgggttttgtagca

SEQ ID NO: 382 - RNA, 21 nt, synthetic construct
  source 1..21: mol_type = other RNA
tgctacaaaacccagaataaa

SEQ ID NO: 383 - RNA, 21 nt, synthetic construct
  source 1..21: mol_type = other RNA
cgttttgcttttgtaacttga

SEQ ID NO: 384 - RNA, 21 nt, synthetic construct
  source 1..21: mol_type = other RNA
tcaagttacaaaagcaaaacg

SEQ ID NO: 385 - RNA, 19 nt, synthetic construct
  source 1..19: mol_type = other RNA
ctttgggtctgtcctctca

SEQ ID NO: 386 - RNA, 21 nt, synthetic construct
  source 1..21: mol_type = other RNA
tgagaggacagacccaaagga

SEQ ID NO: 387 - RNA, 21 nt, synthetic construct
  source 1..21: mol_type = other RNA
ccttttgggtctgtcctctca

SEQ ID NO: 388 - RNA, 21 nt, synthetic construct
  source 1..21: mol_type = other RNA
tgagaggacagacccaaaagg

SEQ ID NO: 389 - RNA, 19 nt, synthetic construct
  source 1..19: mol_type = other RNA
ccttttgggtctgtcctca

SEQ ID NO: 390 - RNA, 21 nt, synthetic construct
  source 1..21: mol_type = other RNA
tgaggacagacccaaaaggta

SEQ ID NO: 391 - RNA, 21 nt, synthetic construct
  source 1..21: mol_type = other RNA
catcttttgggtctgtcctca

SEQ ID NO: 392 - RNA, 21 nt, synthetic construct
  source 1..21: mol_type = other RNA
tgaggacagacccaaaagatg

SEQ ID NO: 393 - RNA, 21 nt, synthetic construct
  source 1..21: mol_type = other RNA
cacatttatcttttgggtcta

SEQ ID NO: 394 - RNA, 21 nt, synthetic construct
  source 1..21: mol_type = other RNA
tagacccaaaagataaatgtg

SEQ ID NO: 395 - RNA, 21 nt, synthetic construct
  source 1..21: mol_type = other RNA
ggacatttatcttttgggtca

SEQ ID NO: 396 - RNA, 21 nt, synthetic construct
  source 1..21: mol_type = other RNA
tgacccaaaagataaatgtcc

SEQ ID NO: 397 - RNA, 19 nt, synthetic construct
  source 1..19: mol_type = other RNA
ggacatttatcttttggga

SEQ ID NO: 398 - RNA, 21 nt, synthetic construct
  source 1..21: mol_type = other RNA
tcccaaaagataaatgtccgc

SEQ ID NO: 399 - RNA, 21 nt, synthetic construct
  source 1..21: mol_type = other RNA
gcggacatttatcttttggga

SEQ ID NO: 400 - RNA, 21 nt, synthetic construct
  source 1..21: mol_type = other RNA
tcccaaaagataaatgtccgc

SEQ ID NO: 401 - RNA, 21 nt, synthetic construct
  source 1..21: mol_type = other RNA
gccctctctgttgccttttta

SEQ ID NO: 402 - RNA, 21 nt, synthetic construct
  source 1..21: mol_type = other RNA
taaaaaggcaacagagagggc

SEQ ID NO: 403 - RNA, 19 nt, synthetic construct
  source 1..19: mol_type = other RNA
actctgggttttgtagcaa

SEQ ID NO: 404 - RNA, 21 nt, synthetic construct
  source 1..21: mol_type = other RNA
ttgctacaaaacccagagtgg

SEQ ID NO: 405 - RNA, 19 nt, synthetic construct
  source 1..19: mol_type = other RNA
ctctgggttttgtagcata

SEQ ID NO: 406 - RNA, 21 nt, synthetic construct
  source 1..21: mol_type = other RNA
tatgctacaaaacccagagtt

SEQ ID NO: 407 - RNA, 19 nt, synthetic construct
  source 1..19: mol_type = other RNA
cctgggttttgtagcatta

SEQ ID NO: 408 - RNA, 21 nt, synthetic construct
  source 1..21: mol_type = other RNA
taatgctacaaaacccaggtt

SEQ ID NO: 409 - RNA, 21 nt, synthetic construct
  source 1..21: mol_type = other RNA
tccagaattgatcaagacaaa

SEQ ID NO: 410 - RNA, 23 nt, synthetic construct
  source 1..23: mol_type = other RNA
tttgtcttgatcaattctggagg

SEQ ID NO: 411 - RNA, 21 nt, synthetic construct
  source 1..21: mol_type = other RNA
ttcctccagaattgatcaaga

SEQ ID NO: 412 - RNA, 23 nt, synthetic construct
  source 1..23: mol_type = other RNA
tcttgatcaattctggaggaaat

SEQ ID NO: 413 - RNA, 21 nt, synthetic construct
  source 1..21: mol_type = other RNA
cagagccaaaatcaagattta

SEQ ID NO: 414 - RNA, 23 nt, synthetic construct
  source 1..23: mol_type = other RNA
taaatcttgattttggctctgga

SEQ ID NO: 415 - RNA, 21 nt, synthetic construct
  source 1..21: mol_type = other RNA
cggagccaaaatcaagattta

SEQ ID NO: 416 - RNA, 23 nt, synthetic construct
  source 1..23: mol_type = other RNA
taaatcttgattttggctttgga

SEQ ID NO: 417 - RNA, 21 nt, synthetic construct
  source 1..21: mol_type = other RNA
cggagccaaaatcaagattta

SEQ ID NO: 418 - RNA, 21 nt, synthetic construct
  source 1..21: mol_type = other RNA
taaatcttgattttggctccg

SEQ ID NO: 419 - RNA, 21 nt, synthetic construct
  source 1..21: mol_type = other RNA
gatcaagacaattcatcatta

SEQ ID NO: 420 - RNA, 23 nt, synthetic construct
  source 1..23: mol_type = other RNA
taatgatgaattgtcttgatcaa

SEQ ID NO: 421 - RNA, 21 nt, synthetic construct
  source 1..21: mol_type = other RNA
tagttatttcctccagaatta

SEQ ID NO: 422 - RNA, 23 nt, synthetic construct
  source 1..23: mol_type = other RNA
taattctggaggaaataactaga

SEQ ID NO: 423 - RNA, 21 nt, synthetic construct
  source 1..21: mol_type = other RNA
aagggccaaattaatgacata

SEQ ID NO: 424 - RNA, 23 nt, synthetic construct
  source 1..23: mol_type = other RNA
tatgtcattaatttggcccttcg

SEQ ID NO: 425 - RNA, 21 nt, synthetic construct
  source 1..21: mol_type = other RNA
aagatttgctatgttagacga

SEQ ID NO: 426 - RNA, 23 nt, synthetic construct
  source 1..23: mol_type = other RNA
tcgtctaacatagcaaatcttga

SEQ ID NO: 427 - RNA, 21 nt, synthetic construct
  source 1..21: mol_type = other RNA
atgttagacgatgtaaaaata

SEQ ID NO: 428 - RNA, 23 nt, synthetic construct
  source 1..23: mol_type = other RNA
tatttttacatcgtctaacatag

SEQ ID NO: 429 - RNA, 21 nt, synthetic construct
  source 1..21: mol_type = other RNA
gactttgtccataagacgaaa

SEQ ID NO: 430 - RNA, 23 nt, synthetic construct
  source 1..23: mol_type = other RNA
tttcgtcttatggacaaagtctt

SEQ ID NO: 431 - RNA, 21 nt, synthetic construct
  source 1..21: mol_type = other RNA
ttgggacatggtcttaaagaa

SEQ ID NO: 432 - RNA, 23 nt, synthetic construct
  source 1..23: mol_type = other RNA
ttctttaagaccatgtcccaact

SEQ ID NO: 433 - RNA, 21 nt, synthetic construct
  source 1..21: mol_type = other RNA
cttaaaacttttgtagaaaaa

SEQ ID NO: 434 - RNA, 23 nt, synthetic construct
  source 1..23: mol_type = other RNA
tttttctacaaaagttttaagtg

SEQ ID NO: 435 - RNA, 21 nt, synthetic construct
  source 1..21: mol_type = other RNA
ctgcaaaccagtgaaatcaaa

SEQ ID NO: 436 - RNA, 23 nt, synthetic construct
  source 1..23: mol_type = other RNA
tttgatttcactggtttgcagcg

SEQ ID NO: 437 - RNA, 21 nt, synthetic construct
  source 1..21: mol_type = other RNA
tttttatgatctatcgctgca

SEQ ID NO: 438 - RNA, 23 nt, synthetic construct
  source 1..23: mol_type = other RNA
tgcagcgatagatcataaaaaga

SEQ ID NO: 439 - RNA, 21 nt, synthetic construct
  source 1..21: mol_type = other RNA
aaccagtgaaatcaaagaaga

SEQ ID NO: 440 - RNA, 23 nt, synthetic construct
  source 1..23: mol_type = other RNA
tcttctttgatttcactggtttg

SEQ ID NO: 441 - RNA, 21 nt, synthetic construct
  source 1..21: mol_type = other RNA
gaccagtgaaatcaaagaaga

SEQ ID NO: 442 - RNA, 23 nt, synthetic construct
  source 1..23: mol_type = other RNA
tcttctttgatttcactggtctg

SEQ ID NO: 443 - RNA, 21 nt, synthetic construct
  source 1..21: mol_type = other RNA
aaccagtgaaatcaaagaaga

SEQ ID NO: 444 - RNA, 21 nt, synthetic construct
  source 1..21: mol_type = other RNA
tcttctttgatttcactggtt

SEQ ID NO: 445 - RNA, 21 nt, synthetic construct
  source 1..21: mol_type = other RNA
gaccagtgaaatcaaagaaga

SEQ ID NO: 446 - RNA, 21 nt, synthetic construct
  source 1..21: mol_type = other RNA
tcttctttgatttcactggtc

SEQ ID NO: 447 - RNA, 21 nt, synthetic construct
  source 1..21: mol_type = other RNA
agaaaaggaactgagaagaaa

SEQ ID NO: 448 - RNA, 23 nt, synthetic construct
  source 1..23: mol_type = other RNA
tttcttctcagttccttttcttc

SEQ ID NO: 449 - RNA, 21 nt, synthetic construct
  source 1..21: mol_type = other RNA
caagtcaaaaatgaagaggta

SEQ ID NO: 450 - RNA, 23 nt, synthetic construct
  source 1..23: mol_type = other RNA
tacctcttcatttttgacttgta

SEQ ID NO: 451 - RNA, 21 nt, synthetic construct
  source 1..21: mol_type = other RNA
taaactacaagtcaaaaatga

SEQ ID NO: 452 - RNA, 23 nt, synthetic construct
  source 1..23: mol_type = other RNA
tcatttttgacttgtagtttata

SEQ ID NO: 453 - RNA, 21 nt, synthetic construct
  source 1..21: mol_type = other RNA
gaggtaaagaatatgtcacta

SEQ ID NO: 454 - RNA, 23 nt, synthetic construct
  source 1..23: mol_type = other RNA
tagtgacatattctttacctctt

SEQ ID NO: 455 - RNA, 21 nt, synthetic construct
  source 1..21: mol_type = other RNA
ggtaaagaatatgtcacttga

SEQ ID NO: 456 - RNA, 23 nt, synthetic construct
  source 1..23: mol_type = other RNA
tcaagtgacatattctttacctc

SEQ ID NO: 457 - RNA, 21 nt, synthetic construct
  source 1..21: mol_type = other RNA
taaagaatatgtcacttgaaa

SEQ ID NO: 458 - RNA, 23 nt, synthetic construct
  source 1..23: mol_type = other RNA
tttcaagtgacatattctttacc

SEQ ID NO: 459 - RNA, 21 nt, synthetic construct
  source 1..21: mol_type = other RNA
ttgaactcaactcaaaactta

SEQ ID NO: 460 - RNA, 23 nt, synthetic construct
  source 1..23: mol_type = other RNA
taagttttgagttgagttcaagt

SEQ ID NO: 461 - RNA, 21 nt, synthetic construct
  source 1..21: mol_type = other RNA
ctgaactcaactcaaaactta

SEQ ID NO: 462 - RNA, 21 nt, synthetic construct
  source 1..21: mol_type = other RNA
taagttttgagttgagttcag

SEQ ID NO: 463 - RNA, 21 nt, synthetic construct
  source 1..21: mol_type = other RNA
tcgaactcaactcaaaactta

SEQ ID NO: 464 - RNA, 21 nt, synthetic construct
  source 1..21: mol_type = other RNA
taagttttgagttgagttcga

SEQ ID NO: 465 - RNA, 21 nt, synthetic construct
  source 1..21: mol_type = other RNA
agaagaaaaaattctacttca

SEQ ID NO: 466 - RNA, 23 nt, synthetic construct
  source 1..23: mol_type = other RNA
tgaagtagaattttttcttctag

SEQ ID NO: 467 - RNA, 21 nt, synthetic construct
  source 1..21: mol_type = other RNA
gaagaaaaaattctacttcaa

SEQ ID NO: 468 - RNA, 23 nt, synthetic construct
  source 1..23: mol_type = other RNA
ttgaagtagaattttttcttcta

SEQ ID NO: 469 - RNA, 21 nt, synthetic construct
  source 1..21: mol_type = other RNA
caaaatcaacctgaaactcca

SEQ ID NO: 470 - RNA, 23 nt, synthetic construct
  source 1..23: mol_type = other RNA
tggagtttcaggttgattttgaa

SEQ ID NO: 471 - RNA, 21 nt, synthetic construct
  source 1..21: mol_type = other RNA
caacctgaaactccagaacaa

SEQ ID NO: 472 - RNA, 23 nt, synthetic construct
  source 1..23: mol_type = other RNA
ttgttctggagtttcaggttgat

SEQ ID NO: 473 - RNA, 21 nt, synthetic construct
  source 1..21: mol_type = other RNA
gaaaaacaagataatagcata

SEQ ID NO: 474 - RNA, 23 nt, synthetic construct
  source 1..23: mol_type = other RNA
tatgctattatcttgtttttcta

SEQ ID NO: 475 - RNA, 21 nt, synthetic construct
  source 1..21: mol_type = other RNA
gaagaccaatataaacaatta

SEQ ID NO: 476 - RNA, 23 nt, synthetic construct
  source 1..23: mol_type = other RNA
taattgtttatattggtcttcca

SEQ ID NO: 477 - RNA, 21 nt, synthetic construct
  source 1..21: mol_type = other RNA
tggaagaccaatataaacaaa

SEQ ID NO: 478 - RNA, 23 nt, synthetic construct
  source 1..23: mol_type = other RNA
tttgtttatattggtcttccacg

SEQ ID NO: 479 - RNA, 21 nt, synthetic construct
  source 1..21: mol_type = other RNA
ctcagaaggactagtattcaa

SEQ ID NO: 480 - RNA, 23 nt, synthetic construct
  source 1..23: mol_type = other RNA
ttgaatactagtccttctgagct

SEQ ID NO: 481 - RNA, 21 nt, synthetic construct
  source 1..21: mol_type = other RNA
agaaggactagtattcaagaa

SEQ ID NO: 482 - RNA, 23 nt, synthetic construct
  source 1..23: mol_type = other RNA
ttcttgaatactagtccttctga

SEQ ID NO: 483 - RNA, 21 nt, synthetic construct
  source 1..21: mol_type = other RNA
atttctctatcttccaagcca

SEQ ID NO: 484 - RNA, 23 nt, synthetic construct
  source 1..23: mol_type = other RNA
tggcttggaagatagagaaattt

SEQ ID NO: 485 - RNA, 21 nt, synthetic construct
  source 1..21: mol_type = other RNA
tttctctatcttccaagccaa

SEQ ID NO: 486 - RNA, 23 nt, synthetic construct
  source 1..23: mol_type = other RNA
ttggcttggaagatagagaaatt

SEQ ID NO: 487 - RNA, 21 nt, synthetic construct
  source 1..21: mol_type = other RNA
cctttcttcagttgaatgaaa

SEQ ID NO: 488 - RNA, 23 nt, synthetic construct
  source 1..23: mol_type = other RNA
tttcattcaactgaagaaaggga

SEQ ID NO: 489 - RNA, 21 nt, synthetic construct
  source 1..21: mol_type = other RNA
gttgaatgaaataagaaatga

SEQ ID NO: 490 - RNA, 23 nt, synthetic construct
  source 1..23: mol_type = other RNA
tcatttcttatttcattcaactg

SEQ ID NO: 491 - RNA, 21 nt, synthetic construct
  source 1..21: mol_type = other RNA
atgtaccaccatttataacaa

SEQ ID NO: 492 - RNA, 23 nt, synthetic construct
  source 1..23: mol_type = other RNA
ttgttataaatggtggtacattc

SEQ ID NO: 493 - RNA, 21 nt, synthetic construct
  source 1..21: mol_type = other RNA
tgtaccaccatttataacaga

SEQ ID NO: 494 - RNA, 23 nt, synthetic construct
  source 1..23: mol_type = other RNA
tctgttataaatggtggtacatt

SEQ ID NO: 495 - RNA, 21 nt, synthetic construct
  source 1..21: mol_type = other RNA
gtccatggacattaattcaaa

SEQ ID NO: 496 - RNA, 23 nt, synthetic construct
  source 1..23: mol_type = other RNA
tttgaattaatgtccatggacta

SEQ ID NO: 497 - RNA, 21 nt, synthetic construct
  source 1..21: mol_type = other RNA
cgtgggagaactacaaatata

SEQ ID NO: 498 - RNA, 23 nt, synthetic construct
  source 1..23: mol_type = other RNA
tatatttgtagttctcccacgtt

SEQ ID NO: 499 - RNA, 21 nt, synthetic construct
  source 1..21: mol_type = other RNA
gttttacgaattgagttggaa

SEQ ID NO: 500 - RNA, 23 nt, synthetic construct
  source 1..23: mol_type = other RNA
ttccaactcaattcgtaaaacat

SEQ ID NO: 501 - RNA, 21 nt, synthetic construct
  source 1..21: mol_type = other RNA
caactatacgctacatctaga

SEQ ID NO: 502 - RNA, 23 nt, synthetic construct
  source 1..23: mol_type = other RNA
tctagatgtagcgtatagttggt

SEQ ID NO: 503 - RNA, 21 nt, synthetic construct
  source 1..21: mol_type = other RNA
tacgctacatctagttgcgaa

SEQ ID NO: 504 - RNA, 23 nt, synthetic construct
  source 1..23: mol_type = other RNA
ttcgcaactagatgtagcgtata

SEQ ID NO: 505 - RNA, 21 nt, synthetic construct
  source 1..21: mol_type = other RNA
tctagttgcgattactggcaa

SEQ ID NO: 506 - RNA, 23 nt, synthetic construct
  source 1..23: mol_type = other RNA
ttgccagtaatcgcaactagatg

SEQ ID NO: 507 - RNA, 21 nt, synthetic construct
  source 1..21: mol_type = other RNA
ctagttgcgattactggcaaa

SEQ ID NO: 508 - RNA, 23 nt, synthetic construct
  source 1..23: mol_type = other RNA
tttgccagtaatcgcaactagat

SEQ ID NO: 509 - RNA, 21 nt, synthetic construct
  source 1..21: mol_type = other RNA
tctacttgggatcacaaagca

SEQ ID NO: 510 - RNA, 23 nt, synthetic construct
  source 1..23: mol_type = other RNA
tgctttgtgatcccaagtagaaa

SEQ ID NO: 511 - RNA, 21 nt, synthetic construct
  source 1..21: mol_type = other RNA
tcttggaagtctcaaaatgga

SEQ ID NO: 512 - RNA, 23 nt, synthetic construct
  source 1..23: mol_type = other RNA
tccattttgagacttccaagata

SEQ ID NO: 513 - RNA, 21 nt, synthetic construct
  source 1..21: mol_type = other RNA
actctataaaatcaaccaaaa

SEQ ID NO: 514 - RNA, 23 nt, synthetic construct
  source 1..23: mol_type = other RNA
ttttggttgattttatagagtat

SEQ ID NO: 515 - RNA, 21 nt, synthetic construct
  source 1..21: mol_type = other RNA
tatcttggaagtctcaaaata

SEQ ID NO: 516 - RNA, 23 nt, synthetic construct
  source 1..23: mol_type = other RNA
tattttgagacttccaagataat

SEQ ID NO: 517 - RNA, 19 nt, synthetic construct
  source 1..19: mol_type = other RNA
catatttgatcagtcttta

SEQ ID NO: 518 - RNA, 21 nt, synthetic construct
  source 1..21: mol_type = other RNA
taaagactgatcaaatatgtt

SEQ ID NO: 519 - RNA, 19 nt, synthetic construct
  source 1..19: mol_type = other RNA
atcaagatttgctatgtta

SEQ ID NO: 520 - RNA, 21 nt, synthetic construct
  source 1..21: mol_type = other RNA
taacatagcaaatcttgattt

SEQ ID NO: 521 - RNA, 19 nt, synthetic construct
  source 1..19: mol_type = other RNA
gtcaagatttgctatgtta

SEQ ID NO: 522 - RNA, 21 nt, synthetic construct
  source 1..21: mol_type = other RNA
taacatagcaaatcttgactt

SEQ ID NO: 523 - RNA, 21 nt, synthetic construct
  source 1..21: mol_type = other RNA
aaatcaagatttgctatgtta

SEQ ID NO: 524 - RNA, 21 nt, synthetic construct
  source 1..21: mol_type = other RNA
taacatagcaaatcttgattt

SEQ ID NO: 525 - RNA, 21 nt, synthetic construct
  source 1..21: mol_type = other RNA
gaatcaagatttgctatgtta

SEQ ID NO: 526 - RNA, 21 nt, synthetic construct
  source 1..21: mol_type = other RNA
taacatagcaaatcttgattc

SEQ ID NO: 527 - RNA, 19 nt, synthetic construct
  source 1..19: mol_type = other RNA
aatcaagatttgctatgta

SEQ ID NO: 528 - RNA, 21 nt, synthetic construct
  source 1..21: mol_type = other RNA
tacatagcaaatcttgatttt

SEQ ID NO: 529 - RNA, 19 nt, synthetic construct
  source 1..19: mol_type = other RNA
gatcaagatttgctatgta

SEQ ID NO: 530 - RNA, 21 nt, synthetic construct
  source 1..21: mol_type = other RNA
tacatagcaaatcttgatctt

SEQ ID NO: 531 - RNA, 21 nt, synthetic construct
  source 1..21: mol_type = other RNA
gaaatcaagatttgctatgta

SEQ ID NO: 532 - RNA, 21 nt, synthetic construct
  source 1..21: mol_type = other RNA
tacatagcaaatcttgatttc

SEQ ID NO: 533 - RNA, 19 nt, synthetic construct
  source 1..19: mol_type = other RNA
aaatcaagatttgctatga

SEQ ID NO: 534 - RNA, 21 nt, synthetic construct
  source 1..21: mol_type = other RNA
tcatagcaaatcttgattttg

SEQ ID NO: 535 - RNA, 19 nt, synthetic construct
  source 1..19: mol_type = other RNA
gaatcaagatttgctatga

SEQ ID NO: 536 - RNA, 21 nt, synthetic construct
  source 1..21: mol_type = other RNA
tcatagcaaatcttgattctg

SEQ ID NO: 537 - RNA, 21 nt, synthetic construct
  source 1..21: mol_type = other RNA
cgaaatcaagatttgctatga

SEQ ID NO: 538 - RNA, 21 nt, synthetic construct
  source 1..21: mol_type = other RNA
tcatagcaaatcttgatttcg

SEQ ID NO: 539 - RNA, 19 nt, synthetic construct
  source 1..19: mol_type = other RNA
aactcaacatatttgatca

SEQ ID NO: 540 - RNA, 21 nt, synthetic construct
  source 1..21: mol_type = other RNA
tgatcaaatatgttgagtttt

SEQ ID NO: 541 - RNA, 19 nt, synthetic construct
  source 1..19: mol_type = other RNA
tttgatcagtctttttata

SEQ ID NO: 542 - RNA, 21 nt, synthetic construct
  source 1..21: mol_type = other RNA
tataaaaagactgatcaaata

SEQ ID NO: 543 - RNA, 19 nt, synthetic construct
  source 1..19: mol_type = other RNA
ccagtgaaatcaaagaaga

SEQ ID NO: 544 - RNA, 21 nt, synthetic construct
  source 1..21: mol_type = other RNA
tcttctttgatttcactggtt

SEQ ID NO: 545 - RNA, 19 nt, synthetic construct
  source 1..19: mol_type = other RNA
gatttgctatgttagacga

SEQ ID NO: 546 - RNA, 21 nt, synthetic construct
  source 1..21: mol_type = other RNA
tcgtctaacatagcaaatctt

SEQ ID NO: 547 - RNA, 21 nt, synthetic construct
  source 1..21: mol_type = other RNA
tcaacatatttgatcagtcta

SEQ ID NO: 548 - RNA, 23 nt, synthetic construct
  source 1..23: mol_type = other RNA
tagactgatcaaatatgttgagt

SEQ ID NO: 549 - RNA, 21 nt, synthetic construct
  source 1..21: mol_type = other RNA
gagccaaaatcaagatttgca

SEQ ID NO: 550 - RNA, 23 nt, synthetic construct
  source 1..23: mol_type = other RNA
tgcaaatcttgattttggctctg

SEQ ID NO: 551 - RNA, 21 nt, synthetic construct
  source 1..21: mol_type = other RNA
ggatagatggatcacaaaaca

SEQ ID NO: 552 - RNA, 23 nt, synthetic construct
  source 1..23: mol_type = other RNA
tgttttgtgatccatctgttcga

SEQ ID NO: 553 - RNA, 21 nt, synthetic construct
  source 1..21: mol_type = other RNA
ggatagatggatcacaaaaca

SEQ ID NO: 554 - RNA, 23 nt, synthetic construct
  source 1..23: mol_type = other RNA
tgttttgtgatccatctgtccga

SEQ ID NO: 555 - RNA, 21 nt, synthetic construct
  source 1..21: mol_type = other RNA
ggatagatggatcacaaaaca

SEQ ID NO: 556 - RNA, 21 nt, synthetic construct
  source 1..21: mol_type = other RNA
tgttttgtgatccatctgtcc

SEQ ID NO: 557 - RNA, 21 nt, synthetic construct
  source 1..21: mol_type = other RNA
cctaaagactttgtccataaa

SEQ ID NO: 558 - RNA, 23 nt, synthetic construct
  source 1..23: mol_type = other RNA
tttatggacaaagtctttaagac

SEQ ID NO: 559 - RNA, 21 nt, synthetic construct
  source 1..21: mol_type = other RNA
cctaaagactttgtccataaa

SEQ ID NO: 560 - RNA, 23 nt, synthetic construct
  source 1..23: mol_type = other RNA
tttatggacaaagtctttaggac

SEQ ID NO: 561 - RNA, 21 nt, synthetic construct
  source 1..21: mol_type = other RNA
cctaaagactttgtccataaa

SEQ ID NO: 562 - RNA, 21 nt, synthetic construct
  source 1..21: mol_type = other RNA
tttatggacaaagtctttagg

SEQ ID NO: 563 - RNA, 21 nt, synthetic construct
  source 1..21: mol_type = other RNA
acatcaggtagtccatggaca

SEQ ID NO: 564 - RNA, 23 nt, synthetic construct
  source 1..23: mol_type = other RNA
tgtccatggactacctgatataa

SEQ ID NO: 565 - RNA, 21 nt, synthetic construct
  source 1..21: mol_type = other RNA
acatcaggtagtccatggaca

SEQ ID NO: 566 - RNA, 23 nt, synthetic construct
  source 1..23: mol_type = other RNA
tgtccatggactacctgatgtaa

SEQ ID NO: 567 - RNA, 21 nt, synthetic construct
  source 1..21: mol_type = other RNA
acatcaggtagtccatggaca

SEQ ID NO: 568 - RNA, 21 nt, synthetic construct
  source 1..21: mol_type = other RNA
tgtccatggactacctgatgt

SEQ ID NO: 569 - RNA, 19 nt, synthetic construct
  source 1..19: mol_type = other RNA
cgcttgaactcaactcaaa

SEQ ID NO: 570 - RNA, 21 nt, synthetic construct
  source 1..21: mol_type = other RNA
tttgagttgagttcaagtggc

SEQ ID NO: 571 - RNA, 21 nt, synthetic construct
  source 1..21: mol_type = other RNA
gccacttgaactcaactcaaa

SEQ ID NO: 572 - RNA, 21 nt, synthetic construct
  source 1..21: mol_type = other RNA
tttgagttgagttcaagtggc

SEQ ID NO: 573 - RNA, 19 nt, synthetic construct
  source 1..19: mol_type = other RNA
cgcttgaactcaactcaaa

SEQ ID NO: 574 - RNA, 21 nt, synthetic construct
  source 1..21: mol_type = other RNA
tttgagttgagttcaagcgac

SEQ ID NO: 575 - RNA, 19 nt, synthetic construct
  source 1..19: mol_type = other RNA
cgcttgaactcaactcaaa

SEQ ID NO: 576 - RNA, 19 nt, synthetic construct
  source 1..19: mol_type = other RNA
tttgagttgagttcaagcg

SEQ ID NO: 577 - RNA, 19 nt, synthetic construct
  source 1..19: mol_type = other RNA
cgcttgaactcaactcaaa

SEQ ID NO: 578 - RNA, 21 nt, synthetic construct
  source 1..21: mol_type = other RNA
tttgagttgagttcaagcggg

SEQ ID NO: 579 - RNA, 19 nt, synthetic construct
  source 1..19: mol_type = other RNA
tacttgaactcaactcaaa

SEQ ID NO: 580 - RNA, 21 nt, synthetic construct
  source 1..21: mol_type = other RNA
tttgagttgagttcaagtggg

SEQ ID NO: 581 - RNA, 19 nt, synthetic construct
  source 1..19: mol_type = other RNA
cactacatataaactacaa

SEQ ID NO: 582 - RNA, 21 nt, synthetic construct
  source 1..21: mol_type = other RNA
ttgtagtttatatgtagtgct

SEQ ID NO: 583 - RNA, 21 nt, synthetic construct
  source 1..21: mol_type = other RNA
ggaactacatataaactacaa

SEQ ID NO: 584 - RNA, 21 nt, synthetic construct
  source 1..21: mol_type = other RNA
ttgtagtttatatgtagttcc

SEQ ID NO: 585 - RNA, 19 nt, synthetic construct
  source 1..19: mol_type = other RNA
cgtataaactacaagtcaa

SEQ ID NO: 586 - RNA, 21 nt, synthetic construct
  source 1..21: mol_type = other RNA
ttgacttgtagtttatgtgta

SEQ ID NO: 587 - RNA, 21 nt, synthetic construct
  source 1..21: mol_type = other RNA
cgcatataaactacaagtcaa

SEQ ID NO: 588 - RNA, 21 nt, synthetic construct
  source 1..21: mol_type = other RNA
ttgacttgtagtttatatgcg

SEQ ID NO: 589 - RNA, 19 nt, synthetic construct
  source 1..19: mol_type = other RNA
ccacaaaacttcaatgaaa

SEQ ID NO: 590 - RNA, 21 nt, synthetic construct
  source 1..21: mol_type = other RNA
tttcattgaagttttgtggtc

SEQ ID NO: 591 - RNA, 21 nt, synthetic construct
  source 1..21: mol_type = other RNA
ggtcacaaaacttcaatgaaa

SEQ ID NO: 592 - RNA, 21 nt, synthetic construct
  source 1..21: mol_type = other RNA
tttcattgaagttttgtgacc

SEQ ID NO: 593 - RNA, 19 nt, synthetic construct
  source 1..19: mol_type = other RNA
ccacaaaacttcaatgaaa

SEQ ID NO: 594 - RNA, 21 nt, synthetic construct
  source 1..21: mol_type = other RNA
tttcattgaagttttgtggtt

SEQ ID NO: 595 - RNA, 19 nt, synthetic construct
  source 1..19: mol_type = other RNA
gggttatactctataaaaa

SEQ ID NO: 596 - RNA, 21 nt, synthetic construct
  source 1..21: mol_type = other RNA
tttttatagagtataactttc

SEQ ID NO: 597 - RNA, 21 nt, synthetic construct
  source 1..21: mol_type = other RNA
ggaggttatactctataaaaa

SEQ ID NO: 598 - RNA, 21 nt, synthetic construct
  source 1..21: mol_type = other RNA
tttttatagagtataacctcc

SEQ ID NO: 599 - RNA, 19 nt, synthetic construct
  source 1..19: mol_type = other RNA
gggaggttatactctataa

SEQ ID NO: 600 - RNA, 21 nt, synthetic construct
  source 1..21: mol_type = other RNA
ttatagagtataacctttcat

SEQ ID NO: 601 - RNA, 21 nt, synthetic construct
  source 1..21: mol_type = other RNA
acggaaggttatactctataa

SEQ ID NO: 602 - RNA, 21 nt, synthetic construct
  source 1..21: mol_type = other RNA
ttatagagtataaccttccgt

SEQ ID NO: 603 - RNA, 19 nt, synthetic construct
  source 1..19: mol_type = other RNA
gcctcaaaatggaaggtta

SEQ ID NO: 604 - RNA, 21 nt, synthetic construct
  source 1..21: mol_type = other RNA
taaccttccattttgaggctt

SEQ ID NO: 605 - RNA, 21 nt, synthetic construct
  source 1..21: mol_type = other RNA
gagtctcaaaatggaaggtta

SEQ ID NO: 606 - RNA, 21 nt, synthetic construct
  source 1..21: mol_type = other RNA
taaccttccattttgagactc

SEQ ID NO: 607 - RNA, 21 nt, synthetic construct
  source 1..21: mol_type = other RNA
gagtctcaaaatggaaggtta

SEQ ID NO: 608 - RNA, 23 nt, synthetic construct
  source 1..23: mol_type = other RNA
taaccttccattttgagactttt

SEQ ID NO: 609 - RNA, 21 nt, synthetic construct
  source 1..21: mol_type = other RNA
gagtctcaaaatggaaggtta

SEQ ID NO: 610 - RNA, 21 nt, synthetic construct
  source 1..21: mol_type = other RNA
taaccttccattttgagactc

SEQ ID NO: 611 - RNA, 21 nt, synthetic construct
  source 1..21: mol_type = other RNA
acggaaggttatactctataa

SEQ ID NO: 612 - RNA, 23 nt, synthetic construct
  source 1..23: mol_type = other RNA
ttatagagtataaccttccgttt

SEQ ID NO: 613 - RNA, 21 nt, synthetic construct
  source 1..21: mol_type = other RNA
acggaaggttatactctataa

SEQ ID NO: 614 - RNA, 21 nt, synthetic construct
  source 1..21: mol_type = other RNA
ttatagagtataaccttccgt

SEQ ID NO: 615 - RNA, 19 nt, synthetic construct
  source 1..19: mol_type = other RNA
gcaaaatgttgatccatca

SEQ ID NO: 616 - RNA, 21 nt, synthetic construct
  source 1..21: mol_type = other RNA
tgatggatcaacattttgctt

SEQ ID NO: 617 - RNA, 21 nt, synthetic construct
  source 1..21: mol_type = other RNA
gaccaaaatgttgatccatca

SEQ ID NO: 618 - RNA, 21 nt, synthetic construct
  source 1..21: mol_type = other RNA
tgatggatcaacattttggtc

SEQ ID NO: 619 - RNA, 21 nt, synthetic construct
  source 1..21: mol_type = other RNA
acgttgatccatccaacagaa

SEQ ID NO: 620 - RNA, 23 nt, synthetic construct
  source 1..23: mol_type = other RNA
ttctgttggatggatcaacgttt

SEQ ID NO: 621 - RNA, 21 nt, synthetic construct
  source 1..21: mol_type = other RNA
acgttgatccatccaacagaa

SEQ ID NO: 622 - RNA, 21 nt, synthetic construct
  source 1..21: mol_type = other RNA
ttctgttggatggatcaacgt

SEQ ID NO: 623 - RNA, 21 nt, synthetic construct
  source 1..21: mol_type = other RNA
gctatactctataaaatcaaa

SEQ ID NO: 624 - RNA, 23 nt, synthetic construct
  source 1..23: mol_type = other RNA
tttgattttatagagtatagcct

SEQ ID NO: 625 - RNA, 21 nt, synthetic construct
  source 1..21: mol_type = other RNA
gctatactctataaaatcaaa

SEQ ID NO: 626 - RNA, 21 nt, synthetic construct
  source 1..21: mol_type = other RNA
tttgattttatagagtatagc

SEQ ID NO: 627 - RNA, 21 nt, synthetic construct
  source 1..21: mol_type = other RNA
gccatactctataaaatcaaa

SEQ ID NO: 628 - RNA, 21 nt, synthetic construct
  source 1..21: mol_type = other RNA
tttgattttatagagtatggc

SEQ ID NO: 629 - RNA, 21 nt, synthetic construct
  source 1..21: mol_type = other RNA
gccatactctataaaatcaaa

SEQ ID NO: 630 - RNA, 23 nt, synthetic construct
  source 1..23: mol_type = other RNA
tttgattttatagagtatggcct

SEQ ID NO: 631 - RNA, 21 nt, synthetic construct
  source 1..21: mol_type = other RNA
gggttatactctataaaatca

SEQ ID NO: 632 - RNA, 23 nt, synthetic construct
  source 1..23: mol_type = other RNA
tgattttatagagtataaccttt

SEQ ID NO: 633 - RNA, 21 nt, synthetic construct
  source 1..21: mol_type = other RNA
gggttatactctataaaatca

SEQ ID NO: 634 - RNA, 21 nt, synthetic construct
  source 1..21: mol_type = other RNA
tgattttatagagtataaccc

SEQ ID NO: 635 - RNA, 19 nt, synthetic construct
  source 1..19: mol_type = other RNA
cgaccaaaatgttgatcca

SEQ ID NO: 636 - RNA, 21 nt, synthetic construct
  source 1..21: mol_type = other RNA
tggatcaacattttggttggt

SEQ ID NO: 637 - RNA, 21 nt, synthetic construct
  source 1..21: mol_type = other RNA
gccaaccaaaatgttgatcca

SEQ ID NO: 638 - RNA, 21 nt, synthetic construct
  source 1..21: mol_type = other RNA
tggatcaacattttggttggc

SEQ ID NO: 639 - RNA, 19 nt, synthetic construct
  source 1..19: mol_type = other RNA
gaatgttgatccatccaaa

SEQ ID NO: 640 - RNA, 21 nt, synthetic construct
  source 1..21: mol_type = other RNA
tttggatggatcaacattctg

SEQ ID NO: 641 - RNA, 21 nt, synthetic construct
  source 1..21: mol_type = other RNA
cgaaatgttgatccatccaaa

SEQ ID NO: 642 - RNA, 21 nt, synthetic construct
  source 1..21: mol_type = other RNA
tttggatggatcaacatttcg

SEQ ID NO: 643 - RNA, 21 nt, synthetic construct
  source 1..21: mol_type = other RNA
cgaccaaaatgttgatccata

SEQ ID NO: 644 - RNA, 23 nt, synthetic construct
  source 1..23: mol_type = other RNA
tatggatcaacattttggttggt

SEQ ID NO: 645 - RNA, 21 nt, synthetic construct
  source 1..21: mol_type = other RNA
cgaccaaaatgttgatccata

SEQ ID NO: 646 - RNA, 21 nt, synthetic construct
  source 1..21: mol_type = other RNA
tatggatcaacattttggtcg

SEQ ID NO: 647 - RNA, 21 nt, synthetic construct
  source 1..21: mol_type = other RNA
cgaccaaaatgttgatccata

SEQ ID NO: 648 - RNA, 23 nt, synthetic construct
  source 1..23: mol_type = other RNA
tatggatcaacattttggtcgat

SEQ ID NO: 649 - RNA, 19 nt, synthetic construct
  source 1..19: mol_type = other RNA
gggaagaactacatataaa

SEQ ID NO: 650 - RNA, 21 nt, synthetic construct
  source 1..21: mol_type = other RNA
tttatatgtagttcttctcgg

SEQ ID NO: 651 - RNA, 21 nt, synthetic construct
  source 1..21: mol_type = other RNA
ccgagaagaactacatataaa

SEQ ID NO: 652 - RNA, 21 nt, synthetic construct
  source 1..21: mol_type = other RNA
tttatatgtagttcttctcgg

SEQ ID NO: 653 - RNA, 21 nt, synthetic construct
  source 1..21: mol_type = other RNA
gtcacaaaacttcaatgaaaa

SEQ ID NO: 654 - RNA, 23 nt, synthetic construct
  source 1..23: mol_type = other RNA
ttttcattgaagttttgtgattt

SEQ ID NO: 655 - RNA, 21 nt, synthetic construct
  source 1..21: mol_type = other RNA
accacaaaacttcaatgaaaa

SEQ ID NO: 656 - RNA, 21 nt, synthetic construct
  source 1..21: mol_type = other RNA
ttttcattgaagttttgtggt

SEQ ID NO: 657 - RNA, 19 nt, synthetic construct
  source 1..19: mol_type = other RNA
cgcaaaacttcaatgaaaa

SEQ ID NO: 658 - RNA, 21 nt, synthetic construct
  source 1..21: mol_type = other RNA
ttttcattgaagttttgcgat

SEQ ID NO: 659 - RNA, 19 nt, synthetic construct
  source 1..19: mol_type = other RNA
cgcaaaacttcaatgaaaa

SEQ ID NO: 660 - RNA, 21 nt, synthetic construct
  source 1..21: mol_type = other RNA
ttttcattgaagttttgtgtt

SEQ ID NO: 661 - RNA, 19 nt, synthetic construct
  source 1..19: mol_type = other RNA
gaacttcaatgaaacgtga

SEQ ID NO: 662 - RNA, 21 nt, synthetic construct
  source 1..21: mol_type = other RNA
tcacgtttcattgaagttctg

SEQ ID NO: 663 - RNA, 21 nt, synthetic construct
  source 1..21: mol_type = other RNA
cgaaacttcaatgaaacgtga

SEQ ID NO: 664 - RNA, 21 nt, synthetic construct
  source 1..21: mol_type = other RNA
tcacgtttcattgaagtttcg

SEQ ID NO: 665 - RNA, 19 nt, synthetic construct
  source 1..19: mol_type = other RNA
ggactcaactcaaaactta

SEQ ID NO: 666 - RNA, 21 nt, synthetic construct
  source 1..21: mol_type = other RNA
taagttttgagttgagttcgg

SEQ ID NO: 667 - RNA, 19 nt, synthetic construct
  source 1..19: mol_type = other RNA
ggactcaactcaaaactta

SEQ ID NO: 668 - RNA, 19 nt, synthetic construct
  source 1..19: mol_type = other RNA
taagttttgagttgagttc

SEQ ID NO: 669 - RNA, 19 nt, synthetic construct
  source 1..19: mol_type = other RNA
gagaatatgtcacttgaaa

SEQ ID NO: 670 - RNA, 21 nt, synthetic construct
  source 1..21: mol_type = other RNA
tttcaagtgacatattctcta

SEQ ID NO: 671 - RNA, 19 nt, synthetic construct
  source 1..19: mol_type = other RNA
ggcaaagaatatgtcacta

SEQ ID NO: 672 - RNA, 21 nt, synthetic construct
  source 1..21: mol_type = other RNA
tagtgacatattctttgcctc

SEQ ID NO: 673 - RNA, 19 nt, synthetic construct
  source 1..19: mol_type = other RNA
ggcaaagaatatgtcacta

SEQ ID NO: 674 - RNA, 19 nt, synthetic construct
  source 1..19: mol_type = other RNA
tagtgacatattctttgcc

SEQ ID NO: 675 - RNA, 19 nt, synthetic construct
  source 1..19: mol_type = other RNA
ggcaaagaatatgtcacta

SEQ ID NO: 676 - RNA, 21 nt, synthetic construct
  source 1..21: mol_type = other RNA
tagtgacatattctttgcctt

SEQ ID NO: 677 - RNA, 19 nt, synthetic construct
  source 1..19: mol_type = other RNA
ggcaaagaatatgtcacta

SEQ ID NO: 678 - RNA, 21 nt, synthetic construct
  source 1..21: mol_type = other RNA
tagtgacatattctttgccgg

SEQ ID NO: 679 - RNA, 21 nt, synthetic construct
  source 1..21: mol_type = other RNA
caggtaaagaatatgtcacta

SEQ ID NO: 680 - RNA, 21 nt, synthetic construct
  source 1..21: mol_type = other RNA
tagtgacatattctttacctg

SEQ ID NO: 681 - RNA, 19 nt, synthetic construct
  source 1..19: mol_type = other RNA
caaagaatatgtcacttga

SEQ ID NO: 682 - RNA, 21 nt, synthetic construct
  source 1..21: mol_type = other RNA
tcaagtgacatattctttgcc

SEQ ID NO: 683 - RNA, 19 nt, synthetic construct
  source 1..19: mol_type = other RNA
caaagaatatgtcacttga

SEQ ID NO: 684 - RNA, 19 nt, synthetic construct
  source 1..19: mol_type = other RNA
tcaagtgacatattctttg

SEQ ID NO: 685 - RNA, 19 nt, synthetic construct
  source 1..19: mol_type = other RNA
gtagatggatcacaaaaca

SEQ ID NO: 686 - RNA, 21 nt, synthetic construct
  source 1..21: mol_type = other RNA
tgttttgtgatccatctactt

SEQ ID NO: 687 - RNA, 19 nt, synthetic construct
  source 1..19: mol_type = other RNA
ccgaatagatggatcacaa

SEQ ID NO: 688 - RNA, 21 nt, synthetic construct
  source 1..21: mol_type = other RNA
ttgtgatccatctattcgggg

SEQ ID NO: 689 - RNA, 19 nt, synthetic construct
  source 1..19: mol_type = other RNA
ctggaagtctcaaaatgga

SEQ ID NO: 690 - RNA, 21 nt, synthetic construct
  source 1..21: mol_type = other RNA
tccattttgagacttccaggg

SEQ ID NO: 691 - RNA, 19 nt, synthetic construct
  source 1..19: mol_type = other RNA
cacttgggatcacaaagca

SEQ ID NO: 692 - RNA, 21 nt, synthetic construct
  source 1..21: mol_type = other RNA
tgctttgtgatcccaagtggg

SEQ ID NO: 693 - RNA, 19 nt, synthetic construct
  source 1..19: mol_type = other RNA
gccatactctataaaatca

SEQ ID NO: 694 - RNA, 21 nt, synthetic construct
  source 1..21: mol_type = other RNA
tgattttatagagtatggctt

SEQ ID NO: 695 - RNA, 19 nt, synthetic construct
  source 1..19: mol_type = other RNA
cgtactctataaaatcaaa

SEQ ID NO: 696 - RNA, 21 nt, synthetic construct
  source 1..21: mol_type = other RNA
tttgattttatagagtacgac

SEQ ID NO: 697 - RNA, 19 nt, synthetic construct
  source 1..19: mol_type = other RNA
gaaaggaactgagaagaaa

SEQ ID NO: 698 - RNA, 21 nt, synthetic construct
  source 1..21: mol_type = other RNA
tttcttctcagttcctttttt

SEQ ID NO: 699 - RNA, 19 nt, synthetic construct
  source 1..19: mol_type = other RNA
gaaaggaactgagaagaaa

SEQ ID NO: 700 - RNA, 19 nt, synthetic construct
  source 1..19: mol_type = other RNA
tttcttctcagttcctttt

SEQ ID NO: 701 - RNA, 19 nt, synthetic construct
  source 1..19: mol_type = other RNA
cccaaaacttgaaagccta

SEQ ID NO: 702 - RNA, 21 nt, synthetic construct
  source 1..21: mol_type = other RNA
taggctttcaagttttgggtt

SEQ ID NO: 703 - RNA, 21 nt, synthetic construct
  source 1..21: mol_type = other RNA
cttacgctgagtacttcgatt

SEQ ID NO: 704 - RNA, 21 nt, synthetic construct
  source 1..21: mol_type = other RNA
tcgaagtactcagcgtaagtt

SEQ ID NO: 705 - DNA, 20 bp, synthetic construct
  source 1..20: mol_type = other DNA
attctgcacaccgagctgaa

SEQ ID NO: 706 - DNA, 24 bp, synthetic construct
  source 1..24: mol_type = other DNA
tcaagctcaaaaaaaatgctgttc

SEQ ID NO: 707 - DNA, 27 bp, synthetic construct
  source 1..27: mol_type = other DNA
ctgcaaaaattgagcaatgaccgcatc

SEQ ID NO: 708 - DNA, 17 bp, synthetic construct
  source 1..17: mol_type = other DNA
acgtggctggcattgca

SEQ ID NO: 709 - DNA, 23 bp, synthetic construct
  source 1..23: mol_type = other DNA
aagtggatcagtctctgcctcaa

SEQ ID NO: 710 - DNA, 22 bp, synthetic construct
  source 1..22: mol_type = other DNA
catgatgctgtctgccgagccg

SEQ ID NO: 711 - DNA, 21 bp, synthetic construct
  source 1..21: mol_type = other DNA
acatgtggctgagattgctgg

SEQ ID NO: 712 - DNA, 24 bp, synthetic construct
  source 1..24: mol_type = other DNA
cctttgctctgtgattccatgtag

SEQ ID NO: 713 - DNA, 28 bp, synthetic construct
  source 1..28: mol_type = other DNA
cctcccagagcacacagacctgatgttt